European Patent Application EP 4 454 706 A1, published October 30, 2024. Title: Novel EGFR antibodies. Applicant: Universität Stuttgart. Application EP. The sequence listing filed with the application follows.

SEQUENCE LISTING (121 sequences)

SEQ ID NO: 1 - protein, 17 aa, synthetic construct
MGDNDIHFAFLSTGAHS

SEQ ID NO: 2 - protein, 20 aa, synthetic construct
METPAQLLFLLLLWLPESTG

SEQ ID NO: 3 - protein, 20 aa, synthetic construct
METDTLLLWVLLLWVPGSTG

SEQ ID NO: 4 - protein, 216 aa, synthetic construct
QPVLTQSPSASGTPGQRVTISCSGVSSNIGRNYVYWYQQFPGTAPKLLIYATHQRPSGVPDRFSGSKSGTSASLAISGLRSEDEANYYCAAWDDGVTGWVFGGGTKLTVLGQPKAAPSVTLFPPSSEELQANKATLVCLISDFYPGAVTVAWKADSSPVKAGVETTTPSKQSNNKYAASSYLSLTPEQWKSHRSYSCQVTHEGSTVEKTVAPTECS

SEQ ID NO: 5 - protein, 239 aa, synthetic construct
QVQLVQSGGGVVQPGGSLRLSCAASGFTFSSYGMHWVRQAPGKGLEWVAFIRYDGSNKYYADSVKGRFTISRDNSKNTLYLQMNSLRAEDTAVYYCAKDGNSGYDSMDYWGQGTLVTVSSASTKGPSVFPLAPSSKSTSGGTAALGCLVKDYFPEPVTVSWNSGALTSGVHTFPAVLQSSGLYSLSSVVTVPSSSLGTQTYICNVNHKPSNTKVDKKVEPKSCGGSGGGGSGGHHHHHH

SEQ ID NO: 6 - protein, 216 aa, synthetic construct
QSVLTQPPSVSGAPGQRVTISCSGGSSNVGRNGVNWFQHLPEKAPKLLIYYDAFLSSGVSDRFSGSKSGTSASLAIRGLQSEDEADYYCASWDDSLTGWVFGGGTKLTVLGQPKAAPSVTLFPPSSEELQANKATLVCLISDFYPGAVTVAWKADSSPVKAGVETTTPSKQSNNKYAASSYLSLTPEQWKSHRSYSCQVTHEGSTVEKTVAPTECS

SEQ ID NO: 7 - protein, 450 aa, synthetic construct
QVQLQESGGGVVQPGGSLRLSCAASGFTFSSYGMHWVRQAPGKGLEWVAFIRYDGSNKYYADSVKGRFTISRDNSKNTLYLQMNSLRAEDTAVYYCAKDGNSGYDSMDYWGQGTLVTVSSASTKGPSVFPLAPSSKSTSGGTAALGCLVKDYFPEPVTVSWNSGALTSGVHTFPAVLQSSGLYSLSSVVTVPSSSLGTQTYICNVNHKPSNTKVDKKVEPKSCDKTHTCPPCPAPELLGGPSVFLFPPKPKDTLMISRTPEVTCVVVDVSHEDPEVKFNWYVDGVEVHNAKTKPREEQYNSTYRVVSVLTVLHQDWLNGKEYKCKVSNKALPAPIEKTISKAKGQPREPQVYTLPPSRDELTKNQVSLTCLVKGFYPSDIAVEWESNGQPENNYKTTPPVLDSDGSFFLYSKLTVDKSRWQQGNVFSCSVMHEALHNHYTQKSLSLSPGK

SEQ ID NO: 8 - protein, 239 aa, synthetic construct
QVQLQESGGGVVQPGGSLRLSCAASGFTFSSYGMHWVRQAPGKGLEWVAFIRYDGSNKYYADSVKGRFTISRDNSKNTLYLQMNSLRAEDTAVYYCAKDGNSGYDSMDYWGQGTLVTVSSASTKGPSVFPLAPSSKSTSGGTAALGCLVKDYFPEPVTVSWNSGALTSGVHTFPAVLQSSGLYSLSSVVTVPSSSLGTQTYICNVNHKPSNTKVDKKVEPKSCGGSGGGGSGGHHHHHH

SEQ ID NO: 9 - protein, 216 aa, synthetic construct
QSVLTQPPSVSGAPGQRVTISCSGGSSNVGRNGVNWFQHLPEKAPKLLIYYDAFLSSGVSDRFSGSKSGTSASLAIRGLQSDDEADYYCAAWDDSLYSWVFGGGTNLTVLGQPKAAPSVTLFPPSSEELQANKATLVCLISDFYPGAVTVAWKADSSPVKAGVETTTPSKQSNNKYAASSYLSLTPEQWKSHRSYSCQVTHEGSTVEKTVAPTECS

SEQ ID NO: 10 - protein, 450 aa, synthetic construct
QVQLVQSGGGVVQPGGSLRLSCAASGFTFSSYGMHWVRQAPGKGLEWVAFIRYDGSNKYYADSVKGRFTISRDNSKNTLYLQMNSLRAEDTAVYYCAKDGNSGYDSMDYWGQGTLVTVSSASTKGPSVFPLAPSSKSTSGGTAALGCLVKDYFPEPVTVSWNSGALTSGVHTFPAVLQSSGLYSLSSVVTVPSSSLGTQTYICNVNHKPSNTKVDKKVEPKSCDKTHTCPPCPAPELLGGPSVFLFPPKPKDTLMISRTPEVTCVVVDVSHEDPEVKFNWYVDGVEVHNAKTKPREEQYNSTYRVVSVLTVLHQDWLNGKEYKCKVSNKALPAPIEKTISKAKGQPREPQVYTLPPSRDELTKNQVSLTCLVKGFYPSDIAVEWESNGQPENNYKTTPPVLDSDGSFFLYSKLTVDKSRWQQGNVFSCSVMHEALHNHYTQKSLSLSPGK

SEQ ID NO: 11 - protein, 452 aa, synthetic construct
EVQLVESGGGVVQPGGSLRLSCAASGFTFSDYDMSWIRQAPGKGLEWVSGILGGSERSYYRDSVKGRFTISRDNSRKTLYLQMNSLRAEDTAVYYCARHGSPGYTLYAWDYWGQGTTVTVSSASTKGPSVFPLAPSSKSTSGGTAALGCLVKDYFPEPVTVSWNSGALTSGVHTFPAVLQSSGLYSLSSVVTVPSSSLGTQTYICNVNHKPSNTKVDKKVEPKSCDKTHTCPPCPAPELLGGPSVFLFPPKPKDTLMISRTPEVTCVVVDVSHEDPEVKFNWYVDGVEVHNAKTKPREEQYNSTYRVVSVLTVLHQDWLNGKEYKCKVSNKALPAPIEKTISKAKGQPREPQVYTLPPSREEMTKNQVSLTCLVKGFYPSDIAVEWESNGQPENNYKTTPPVLDSDGSFFLYSKLTVDKSRWQQGNVFSCSVMHEALHNHYTQKSLSLSPGK

SEQ ID NO: 12 - protein, 219 aa, synthetic construct
DIVMTQTPLSLPVTPGEPASISCRSNQDLTHSNGNTYLEWYLQKPGQSPRLLIYKVSNRFSGVPDRFSGSGAGTDFTLRISRVEAEDVGVYYCMQGTHWPWTFGQGTKVDIKRTVAAPSVFIFPPSDEQLKSGTASVVCLLNNFYPREAKVQWKVDNALQSGNSQESVTEQDSKDSTYSLSSTLTLSKADYEKHKVYACEVTHQGLSSPVTKSFNRGEC

SEQ ID NO: 13 - protein, 451 aa, synthetic construct
QVQLVQSGAEVKKPGASVKVSCKASGYTFTSHWMHWVRQAPGQGLEWIGEFNPSNGRTNYNEKFKSKATMTVDTSTNTAYMELSSLRSEDTAVYYCASRDYDYDGRYFDYWGQGTLVTVSSASTKGPSVFPLAPSSKSTSGGTAALGCLVKDYFPEPVTVSWNSGALTSGVHTFPAVLQSSGLYSLSSVVTVPSSSLGTQTYICNVNHKPSNTKVDKKVEPKSCDKTHTCPPCPAPELLGGPSVFLFPPKPKDTLMISRTPEVTCVVVDVSHEDPEVKFNWYVDGVEVHNAKTKPREEQYNSTYRVVSVLTVLHQDWLNGKEYKCKVSNKALPAPIEKTISKAKGQPREPQVYTLPPSREEMTKNQVSLTCLVKGFYPSDIAVEWESNGQPENNYKTTPPVLDSDGSFFLYSKLTVDKSRWQQGNVFSCSVMHEALHNHYTQKSLSLSPGK

SEQ ID NO: 14 - protein, 213 aa, synthetic construct
DIQMTQSPSSLSASVGDRVTITCSASSSVTYMYWYQQKPGKAPKLLIYDTSNLASGVPSRFSGSGSGTDYTFTISSLQPEDIATYYCQQWSSHIFTFGQGTKVEIKRTVAAPSVFIFPPSDEQLKSGTASVVCLLNNFYPREAKVQWKVDNALQSGNSQESVTEQDSKDSTYSLSSTLTLSKADYEKHKVYACEVTHQGLSSPVTKSFNRGEC

SEQ ID NO: 15 - protein, 451 aa, synthetic construct
QVQLQESGPGLVKPSQTLSLTCTVSGGSISSGDYYWSWIRQPPGKGLEWIGYIYYSGSTDYNPSLKSRVTMSVDTSKNQFSLKVNSVTAADTAVYYCARVSIFGVGTFDYWGQGTLVTVSSASTKGPSVFPLAPSSKSTSGGTAALGCLVKDYFPEPVTVSWNSGALTSGVHTFPAVLQSSGLYSLSSVVTVPSSSLGTQTYICNVNHKPSNTKVDKKVEPKSCDKTHTCPPCPAPELLGGPSVFLFPPKPKDTLMISRTPEVTCVVVDVSHEDPEVKFNWYVDGVEVHNAKTKPREEQYNSTYRVVSVLTVLHQDWLNGKEYKCKVSNKALPAPIEKTISKAKGQPREPQVYTLPPSREEMTKNQVSLTCLVKGFYPSDIAVEWESNGQPENNYKTTPPVLDSDGSFFLYSKLTVDKSRWQQGNVFSCSVMHEALHNHYTQKSLSLSPGK

SEQ ID NO: 16 - protein, 214 aa, synthetic construct
EIVMTQSPATLSLSPGERATLSCRASQSVSSYLAWYQQKPGQAPRLLIYDASNRATGIPARFSGSGSGTDFTLTISSLEPEDFAVYYCHQYGSTPLTFGGGTKAEIKRTVAAPSVFIFPPSDEQLKSGTASVVCLLNNFYPREAKVQWKVDNALQSGNSQESVTEQDSKDSTYSLSSTLTLSKADYEKHKVYACEVTHQGLSSPVTKSFNRGEC

SEQ ID NO: 17 - protein, 449 aa, synthetic construct
QVQLQESGPGLVKPSETLSLTCTVSGGSVSSGDYYWTWIRQSPGKGLEWIGHIYYSGNTNYNPSLKSRLTISIDTSKTQFSLKLSSVTAADTAIYYCVRDRVTGAFDIWGQGTMVTVSSASTKGPSVFPLAPSSKSTSGGTAALGCLVKDYFPEPVTVSWNSGALTSGVHTFPAVLQSSGLYSLSSVVTVPSSSLGTQTYICNVNHKPSNTKVDKKVEPKSCDKTHTCPPCPAPELLGGPSVFLFPPKPKDTLMISRTPEVTCVVVDVSHEDPEVKFNWYVDGVEVHNAKTKPREEQYNSTYRVVSVLTVLHQDWLNGKEYKCKVSNKALPAPIEKTISKAKGQPREPQVYTLPPSREEMTKNQVSLTCLVKGFYPSDIAVEWESNGQPENNYKTTPPVLDSDGSFFLYSKLTVDKSRWQQGNVFSCSVMHEALHNHYTQKSLSLSPGK

SEQ ID NO: 18 - protein, 214 aa, synthetic construct
DIQMTQSPSSLSASVGDRVTITCQASQDISNYLNWYQQKPGKAPKLLIYDASNLETGVPSRFSGSGSGTDFTFTISSLQPEDIATYFCQHFDHLPLAFGGGTKVEIKRTVAAPSVFIFPPSDEQLKSGTASVVCLLNNFYPREAKVQWKVDNALQSGNSQESVTEQDSKDSTYSLSSTLTLSKADYEKHKVYACEVTHQGLSSPVTKSFNRGEC

SEQ ID NO: 19 - protein, 512 aa, synthetic construct
QVQLVQSGGGVVQPGGSLRLSCAASGFTFSSYGMHWVRQAPGKGLEWVAFIRYDGSNKYYADSVKGRFTISRDNSKNTLYLQMNSLRAEDTAVYYCAKDGNSGYDSMDYWGQGTLVTVSSGGGGSDIQMTQSPSSLSASVGDRVTITCRASQDIRNYLNWYQQKPGKAPKLLIYYTSRLHSGVPSRFSGSGSGTDFTFTISSLQPEDIATYYCQQGNTLPWTFGQGTKLEIKRGGGGSGGGGSGGGGSQVQLVQSGAEVKKPGSSVKVSCKASGGTFSGYTMNWVRQAPGQGLEWMGLINPYKGVSTYNGKFKDRVTITADKSTSTAYMELSSLRSEDTAVYYCARSGYYGDSDWYFDVWGQGTLVTVSSGGGGSQSVLTQPPSVSGAPGQRVTISCSGGSSNVGRNGVNWFQHLPEKAPKLLIYYDAFLSSGVSDRFSGSKSGTSASLAIRGLQSDDEADYYCAAWDDSLYSWVFGGGTNLTVLAAAGGSGGGGSGGGTGGGGSLHHHHHH

SEQ ID NO: 20 - protein, 754 aa, synthetic construct
QVQLVQSGGGVVQPGGSLRLSCAASGFTFSSYGMHWVRQAPGKGLEWVAFIRYDGSNKYYADSVKGRFTISRDNSKNTLYLQMNSLRAEDTAVYYCAKDGNSGYDSMDYWGQGTLVTVSSGGGGSDIQMTQSPSSLSASVGDRVTITCRASQDIRNYLNWYQQKPGKAPKLLIYYTSRLHSGVPSRFSGSGSGTDFTFTISSLQPEDIATYYCQQGNTLPWTFGQGTKLEIKRGGGGSGGGGSGGGGSQVQLVQSGAEVKKPGSSVKVSCKASGGTFSGYTMNWVRQAPGQGLEWMGLINPYKGVSTYNGKFKDRVTITADKSTSTAYMELSSLRSEDTAVYYCARSGYYGDSDWYFDVWGQGTLVTVSSGGGGSQSVLTQPPSVSGAPGQRVTISCSGGSSNVGRNGVNWFQHLPEKAPKLLIYYDAFLSSGVSDRFSGSKSGTSASLAIRGLQSDDEADYYCAAWDDSLYSWVFGGGTNLTVLAAAGGSGGGGSGGGTQVQLVQSGGGVVQPGGSLRLSCAASGFTFSSYGMHWVRQAPGKGLEWVAFIRYDGSNKYYADSVKGRFTISRDNSKNTLYLQMNSLRAEDTAVYYCAKDGNSGYDSMDYWGQGTLVTVSSGGGGSGGGGSGGGGSQSVLTQPPSVSGAPGQRVTISCSGGSSNVGRNGVNWFQHLPEKAPKLLIYYDAFLSSGVSDRFSGSKSGTSASLAIRGLQSDDEADYYCAAWDDSLYSWVFGGGTNLTVLGSLHHHHHH

SEQ ID NO: 21 - protein, 451 aa, synthetic construct
QVQLVQSGGGVVQPGGSLRLSCAASGFTFSSYGMHWVRQAPGKGLEWVAFIRYDGSNKYYADSVKGRFTISRDNSKNTLYLQMNSLRAEDTAVYYCAKDGNSGYDSMDYWGQGTLVTVSSASTKGPSVFPLAPSSKSTSGGTAALGCLVKDYFPEPVTVSWNSGALTSGVHTFPAVLQSSGLYSLSSVVTVPSSSLGTQTYICNVNHKPSNTKVDKKVEPKSCGTDKTHTCPPCPAPPVAGPSVFLFPPKPKDTLMISRTPEVTCVVVDVSHEDPEVKFNWYVDGVEVHNAKTKPREEQYNSTYRVVSVLTVLHQDWLNGKEYKCKVSNKGLPSSIEKTISKAKGQPREPQVCTLPPSRDELTKNQVSLSCAVKGFYPSDIAVEWESNGQPENNYKTTPPVLDSDGSFFLVSKLTVDKSRWQQGNVFSCSVMHEALHNHYTQKSLSLSPGK

SEQ ID NO: 22 - protein, 689 aa, synthetic construct
QVQLVQSGGGVVQPGGSLRLSCAASGFTFSSYGMHWVRQAPGKGLEWVAFIRYDGSNKYYADSVKGRFTISRDNSKNTLYLQMNSLRAEDTAVYYCAKDGNSGYDSMDYWGQGTLVTVSSASTKGPSVFPLAPSSKSTSGGTAALGCLVKDYFPEPVTVSWNSGALTSGVHTFPAVLQSSGLYSLSSVVTVPSSSLGTQTYICNVNHKPSNTKVDKKVEPKSCGGSGGGGSGGQVQLVQSGAEVKKPGSSVKVSCKASGGTFSGYTMNWVRQAPGQGLEWMGLINPYKGVSTYNGKFKDRVTITADKSTSTAYMELSSLRSEDTAVYYCARSGYYGDSDWYFDVWGQGTLVTVSSDFTPPTVKILQSSCDGGGHFPPTIQLLCLVSGYTPGTINITWLEDGQVMDVDLSTASTTQEGELASTQSELTLSQKHWLSDRTYTCQVTYQGHTFEDSTKKSADSNGTDKTHTCPPCPAPPVAGPSVFLFPPKPKDTLMISRTPEVTCVVVDVSHEDPEVKFNWYVDGVEVHNAKTKPREEQYNSTYRVVSVLTVLHQDWLNGKEYKCKVSNKGLPSSIEKTISKAKGQPREPQVYTLPPCRDELTKNQVSLWCLVKGFYPSDIAVEWESNGQPENNYKTTPPVLDSDGSFFLYSKLTVDKSRWQQGNVFSCSVMHEALHNHYTQKSLSLSPGK

SEQ ID NO: 23 - protein, 456 aa, synthetic construct
QVQLVQSGAEVKKPGSSVKVSCKASGGTFSGYTMNWVRQAPGQGLEWMGLINPYKGVSTYNGKFKDRVTITADKSTSTAYMELSSLRSEDTAVYYCARSGYYGDSDWYFDVWGQGTLVTVSSDFTPPTVKILQSSCDGGGHFPPTIQLLCLVSGYTPGTINITWLEDGQVMDVDLSTASTTQEGELASTQSELTLSQKHWLSDRTYTCQVTYQGHTFEDSTKKSADSNGTDKTHTCPPCPAPPVAGPSVFLFPPKPKDTLMISRTPEVTCVVVDVSHEDPEVKFNWYVDGVEVHNAKTKPREEQYNSTYRVVSVLTVLHQDWLNGKEYKCKVSNKGLPSSIEKTISKAKGQPREPQVYTLPPCRDELTKNQVSLWCLVKGFYPSDIAVEWESNGQPENNYKTTPPVLDSDGSFFLYSKLTVDKSRWQQGNVFSCSVMHEALHNHYTQKSLSLSPGK

SEQ ID NO: 24 - protein, 215 aa, synthetic construct
DIQMTQSPSSLSASVGDRVTITCRASQDIRNYLNWYQQKPGKAPKLLIYYTSRLHSGVPSRFSGSGSGTDFTFTISSLQPEDIATYYCQQGNTLPWTFGQGTKLEIKRTDFTPPTVKILQSSSDGGGHFPPTIQLLCLVSGYTPGTIQITWLEDGQVMDVDLSTASTTQEGELASTQSELTLSQKHWLSDRTYTCQVTYQGHTFEDSTKKCADSN

SEQ ID NO: 25 - protein, 214 aa, synthetic construct
DIQMTQSPSSLPASLGDRVTINCQASQDISNYLNWYQQKPGKAPKLLIYYTNKLADGVPSRFSGSGSGRDSSFTISSLESEDIGSYYCQQYYNYPWTFGPGTKLEIKRTVAAPSVFIFPPSDEQLKSGTASVVCLLNNFYPREAKVQWKVDNALQSGNSQESVTEQDSKDSTYSLSSTLTLSKADYEKHKVYACEVTHQGLSSPVTKSFNRGEC

SEQ ID NO: 26 - protein, 454 aa, synthetic construct
QVQLVQSGGGVVQPGGSLRLSCAASGFTFSSYGMHWVRQAPGKGLEWVAFIRYDGSNKYYADSVKGRFTISRDNSKNTLYLQMNSLRAEDTAVYYCAKDGNSGYDSMDYWGQGTLVTVSSDFTPPTVKILQSSCDGGGHFPPTIQLLCLVSGYTPGTINITWLEDGQVMDVDLSTASTTQEGELASTQSELTLSQKHWLSDRTYTCQVTYQGHTFEDSTKKSADSNGTDKTHTCPPCPAPPVAGPSVFLFPPKPKDTLMISRTPEVTCVVVDVSHEDPEVKFNWYVDGVEVHNAKTKPREEQYNSTYRVVSVLTVLHQDWLNGKEYKCKVSNKGLPSSIEKTISKAKGQPREPQVCTLPPSRDELTKNQVSLSCAVKGFYPSDIAVEWESNGQPENNYKTTPPVLDSDGSFFLVSKLTVDKSRWQQGNVFSCSVMHEALHNHYTQKSLSLSPGK

SEQ ID NO: 27 - protein, 216 aa, synthetic construct
QSVLTQPPSVSGAPGQRVTISCSGGSSNVGRNGVNWFQHLPEKAPKLLIYYDAFLSSGVSDRFSGSKSGTSASLAIRGLQSDDEADYYCAAWDDSLYSWVFGGGTNLTVLDFTPPTVKILQSSSDGGGHFPPTIQLLCLVSGYTPGTIQITWLEDGQVMDVDLSTASTTQEGELASTQSELTLSQKHWLSDRTYTCQVTYQGHTFEDSTKKCADSN

SEQ ID NO: 28 - protein, 447 aa, synthetic construct
EVQLVESGGGLVQPGKSLKLSCEASGFTFSGYGMHWVRQAPGRGLESVAYITSSSINIKYADAVKGRFTVSRDNAKNLLFLQMNILKSEDTAMYYCARFDWDKNYWGQGTMVTVSSASTKGPSVFPLAPSSKSTSGGTAALGCLVKDYFPEPVTVSWNSGALTSGVHTFPAVLQSSGLYSLSSVVTVPSSSLGTQTYICNVNHKPSNTKVDKKVEPKSCGTDKTHTCPPCPAPPVAGPSVFLFPPKPKDTLMISRTPEVTCVVVDVSHEDPEVKFNWYVDGVEVHNAKTKPREEQYNSTYRVVSVLTVLHQDWLNGKEYKCKVSNKGLPSSIEKTISKAKGQPREPQVYTLPPCRDELTKNQVSLWCLVKGFYPSDIAVEWESNGQPENNYKTTPPVLDSDGSFFLYSKLTVDKSRWQQGNVFSCSVMHEALHNHYTQKSLSLSPGK

SEQ ID NO: 29 - protein, 683 aa, synthetic construct
QVQLVQSGGGVVQPGGSLRLSCAASGFTFSSYGMHWVRQAPGKGLEWVAFIRYDGSNKYYADSVKGRFTISRDNSKNTLYLQMNSLRAEDTAVYYCAKDGNSGYDSMDYWGQGTLVTVSSDFTPPTVKILQSSCDGGGHFPPTIQLLCLVSGYTPGTINITWLEDGQVMDVDLSTASTTQEGELASTQSELTLSQKHWLSDRTYTCQVTYQGHTFEDSTKKSADSNGGSGGGGSGGEVQLVESGGGLVQPGKSLKLSCEASGFTFSGYGMHWVRQAPGRGLESVAYITSSSINIKYADAVKGRFTVSRDNAKNLLFLQMNILKSEDTAMYYCARFDWDKNYWGQGTMVTVSSASTKGPSVFPLAPSSKSTSGGTAALGCLVKDYFPEPVTVSWNSGALTSGVHTFPAVLQSSGLYSLSSVVTVPSSSLGTQTYICNVNHKPSNTKVDKKVEPKSCGTDKTHTCPPCPAPPVAGPSVFLFPPKPKDTLMISRTPEVTCVVVDVSHEDPEVKFNWYVDGVEVHNAKTKPREEQYNSTYRVVSVLTVLHQDWLNGKEYKCKVSNKGLPSSIEKTISKAKGQPREPQVYTLPPCRDELTKNQVSLWCLVKGFYPSDIAVEWESNGQPENNYKTTPPVLDSDGSFFLYSKLTVDKSRWQQGNVFSCSVMHEALHNHYTQKSLSLSPGK

SEQ ID NO: 30 - protein, 450 aa, synthetic construct
QVQLKQSGPGLVQPSQSLSITCTVSGFSLTNYGVHWVRQSPGKGLEWLGVIWSGGNTDYNTPFTSRLSINKDNSKSQVFFKMNSLQSNDTAIYYCARALTYYDYEFAYWGQGTLVTVSAASTKGPSVFPLAPSSKSTSGGTAALGCLVKDYFPEPVTVSWNSGALTSGVHTFPAVLQSSGLYSLSSVVTVPSSSLGTQTYICNVNHKPSNTKVDKKVEPKSCGTDKTHTCPPCPAPPVAGPSVFLFPPKPKDTLMISRTPEVTCVVVDVSHEDPEVKFNWYVDGVEVHNAKTKPREEQYNSTYRVVSVLTVLHQDWLNGKEYKCKVSNKGLPSSIEKTISKAKGQPREPQVCTLPPSRDELTKNQVSLSCAVKGFYPSDIAVEWESNGQPENNYKTTPPVLDSDGSFFLVSKLTVDKSRWQQGNVFSCSVMHEALHNHYTQKSLSLSPGK

SEQ ID NO: 31 - protein, 688 aa, synthetic construct
QVQLKQSGPGLVQPSQSLSITCTVSGFSLTNYGVHWVRQSPGKGLEWLGVIWSGGNTDYNTPFTSRLSINKDNSKSQVFFKMNSLQSNDTAIYYCARALTYYDYEFAYWGQGTLVTVSAASTKGPSVFPLAPSSKSTSGGTAALGCLVKDYFPEPVTVSWNSGALTSGVHTFPAVLQSSGLYSLSSVVTVPSSSLGTQTYICNVNHKPSNTKVDKKVEPKSCGGSGGGGSGGQVQLVQSGAEVKKPGSSVKVSCKASGGTFSGYTMNWVRQAPGQGLEWMGLINPYKGVSTYNGKFKDRVTITADKSTSTAYMELSSLRSEDTAVYYCARSGYYGDSDWYFDVWGQGTLVTVSSDFTPPTVKILQSSCDGGGHFPPTIQLLCLVSGYTPGTINITWLEDGQVMDVDLSTASTTQEGELASTQSELTLSQKHWLSDRTYTCQVTYQGHTFEDSTKKSADSNGTDKTHTCPPCPAPPVAGPSVFLFPPKPKDTLMISRTPEVTCVVVDVSHEDPEVKFNWYVDGVEVHNAKTKPREEQYNSTYRVVSVLTVLHQDWLNGKEYKCKVSNKGLPSSIEKTISKAKGQPREPQVYTLPPCRDELTKNQVSLWCLVKGFYPSDIAVEWESNGQPENNYKTTPPVLDSDGSFFLYSKLTVDKSRWQQGNVFSCSVMHEALHNHYTQKSLSLSPGK

SEQ ID NO: 32 - protein, 214 aa, synthetic construct
DILLTQSPVILSVSPGERVSFSCRASQSIGTNIHWYQQRTNGSPRLLIKYASESISGIPSRFSGSGSGTDFTLSINSVESEDIADYYCQQNNNWPTTFGAGTKLELKRTVAAPSVFIFPPSDEQLKSGTASVVCLLNNFYPREAKVQWKVDNALQSGNSQESVTEQDSKDSTYSLSSTLTLSKADYEKHKVYACEVTHQGLSSPVTKSFNRGEC

SEQ ID NO: 33 - protein, 854 aa, synthetic construct
DAAQPALEEKKVCQGTSNKLTQLGTFEDHFLSLQRMFNNCEVVLGNLEITYVQRNYDLSFLKTIQEVAGYVLIALNTVERIPLENLQIIRGNMYYENSYALAVLSNYDANKTGLKELPMRNLQEILHGAVRFSNNPALCNVESIQWRDIVSSDFLSNMSMDFQNHLGSCQKCDPSCPNGSCWGAGEENCQKLTKIICAQQCSGRCRGKSPSDCCHNQCAAGCTGPRESDCLVCRKFRDEATCKDTCPPLMLYNPTTYQMDVNPEGKYSFGATCVKKCPRNYVVTDHGSCVRACGADSYEMEEDGVRKCKKCEGPCRKVCNGIGIGEFKDSLSINATNIKHFKNCTSISGDLHILPVAFRGDSFTHTPPLDPQELDILKTVKEITGFLLIQAWPENRTDLHAFENLEIIRGRTKQHGQFSLAVVSLNITSLGLRSLKEISDGDVIISGNKNLCYANTINWKKLFGTSGQKTKIISNRGENSCKATGQVCHALCSPEGCWGPEPRDCVSCRNVSRGRECVDKCNLLEGEPREFVENSECIQCHPECLPQAMNITCTGRGPDNCIQCAHYIDGPHCVKTCPAGVMGENNTLVWKYADAGHVCHLCHPNCTYGCTGPGLEGCPTNGPKIPSAAASPPCKCPAPNLLGGPSVFIFPPKIKDVLMISLSPIVTCVVVDVSEDDPDVQISWFVNNVEVHTAQTQTHREDYNSTLRVVSALPIQHQDWMSGKEFKCKVNNKDLPAPIERTISKPKGSVRAPQVYVLPPPEEEMTKKQVTLTCMVTDFMPEDIYVEWTNNGKTELNYKNTEPVLDSDGSYFMYSKLRVEKKNWVERNSYSCSVVHEGLHNHHTTKSFSRTPGK

SEQ ID NO: 34 - protein, 854 aa, synthetic construct
DAAQPALEEKKVCQGTSNKLTQLGTFEDHFLSLQRMFNNCEVVLGNLEITYVQRNYDLSFLKTIQEVAGYVLIALNTVERIPLENLQIIRGNMYYENSYALAVLSNYDANKTGLKELPMRNLQEILHGAVRFSNNPALCNVESIQWRDIVSSDFLSNMSMDFQNHLGSCQKCDPSCPNGSCWGAGEENCQKLTKIICAQQCSGRCRGKSPSDCCHNQCAAGCTGPRESDCLVCRKFRDEATCKDTCPPLMLYNPTTYQMDVNPEGKYSFGATCVKKCPRNYVVTDHGSCVRACGADSYEMEEDGVRKCKKCEGPCRKVCNGIGIGEFKDSLSINATNIKHFKNCTSISGDLHILPVAFRGDSFTHTPPLDPQELDILKTVKEITGFLLIQAWPENRTDLHAFENLEIIRGRTKQHAQFSLAVVSLNITSLGLRSLKEISDGDVIISGNKNLCYANTINWKKLFGTSGQKTKIISNRGENSCKATGQVCHALCSPEGCWGPEPRDCVSCRNVSRGRECVDKCNLLEGEPREFVENSECIQCHPECLPQAMNITCTGRGPDNCIQCAHYIDGPHCVKTCPAGVMGENNTLVWKYADAGHVCHLCHPNCTYGCTGPGLEGCPTNGPKIPSAAASPPCKCPAPNLLGGPSVFIFPPKIKDVLMISLSPIVTCVVVDVSEDDPDVQISWFVNNVEVHTAQTQTHREDYNSTLRVVSALPIQHQDWMSGKEFKCKVNNKDLPAPIERTISKPKGSVRAPQVYVLPPPEEEMTKKQVTLTCMVTDFMPEDIYVEWTNNGKTELNYKNTEPVLDSDGSYFMYSKLRVEKKNWVERNSYSCSVVHEGLHNHHTTKSFSRTPGK

SEQ ID NO: 35 - protein, 854 aa, synthetic construct
DAAQPALEEKKVCQGTSNKLTQLGTFEDHFLSLQRMFNNCEVVLGNLEITYVQRNYDLSFLKTIQEVAGYVLIALNTVERIPLENLQIIRGNMYYENSYALAVLSNYDANKTGLKELPMRNLQEILHGAVRFSNNPALCNVESIQWRDIVSSDFLSNMSMDFQNHLGSCQKCDPSCPNGSCWGAGEENCQKLTKIICAQQCSGRCRGKSPSDCCHNQCAAGCTGPRESDCLVCRKFRDEATCKDTCPPLMLYNPTTYQMDVNPEGKYSFGATCVKKCPRNYVVTDHGSCVRACGADSYEMEEDGVRKCKKCEGPCRKVCNGIGIGEFKDSLSINATNIKHFKNCTSISGDLHILPVAFRGDSFTHTPPLDPQELDILKTVKEITGFLLIQAWPENRTDLHAFENLEIIRGRTKQHGPFSLAVVSLNITSLGLRSLKEISDGDVIISGNKNLCYANTINWKKLFGTSGQKTKIISNRGENSCKATGQVCHALCSPEGCWGPEPRDCVSCRNVSRGRECVDKCNLLEGEPREFVENSECIQCHPECLPQAMNITCTGRGPDNCIQCAHYIDGPHCVKTCPAGVMGENNTLVWKYADAGHVCHLCHPNCTYGCTGPGLEGCPTNGPKIPSAAASPPCKCPAPNLLGGPSVFIFPPKIKDVLMISLSPIVTCVVVDVSEDDPDVQISWFVNNVEVHTAQTQTHREDYNSTLRVVSALPIQHQDWMSGKEFKCKVNNKDLPAPIERTISKPKGSVRAPQVYVLPPPEEEMTKKQVTLTCMVTDFMPEDIYVEWTNNGKTELNYKNTEPVLDSDGSYFMYSKLRVEKKNWVERNSYSCSVVHEGLHNHHTTKSFSRTPGK

SEQ ID NO: 36 - protein, 854 aa, synthetic construct
DAAQPALEEKKVCQGTSNKLTQLGTFEDHFLSLQRMFNNCEVVLGNLEITYVQRNYDLSFLKTIQEVAGYVLIALNTVERIPLENLQIIRGNMYYENSYALAVLSNYDANKTGLKELPMRNLQEILHGAVRFSNNPALCNVESIQWRDIVSSDFLSNMSMDFQNHLGSCQKCDPSCPNGSCWGAGEENCQKLTKIICAQQCSGRCRGKSPSDCCHNQCAAGCTGPRESDCLVCRKFRDEATCKDTCPPLMLYNPTTYQMDVNPEGKYSFGATCVKKCPRNYVVTDHGSCVRACGADSYEMEEDGVRKCKKCEGPCRKVCNGIGIGEFKDSLSINATNIKHFKNCTSISGDLHILPVAFRGDSFTHTPPLDPQELDILKTVKEITGFLLIQAWPENRTDLHAFENLEIIRGRTKQHGQASLAVVSLNITSLGLRSLKEISDGDVIISGNKNLCYANTINWKKLFGTSGQKTKIISNRGENSCKATGQVCHALCSPEGCWGPEPRDCVSCRNVSRGRECVDKCNLLEGEPREFVENSECIQCHPECLPQAMNITCTGRGPDNCIQCAHYIDGPHCVKTCPAGVMGENNTLVWKYADAGHVCHLCHPNCTYGCTGPGLEGCPTNGPKIPSAAASPPCKCPAPNLLGGPSVFIFPPKIKDVLMISLSPIVTCVVVDVSEDDPDVQISWFVNNVEVHTAQTQTHREDYNSTLRVVSALPIQHQDWMSGKEFKCKVNNKDLPAPIERTISKPKGSVRAPQVYVLPPPEEEMTKKQVTLTCMVTDFMPEDIYVEWTNNGKTELNYKNTEPVLDSDGSYFMYSKLRVEKKNWVERNSYSCSVVHEGLHNHHTTKSFSRTPGK

SEQ ID NO: 37 - protein, 854 aa, synthetic construct
DAAQPALEEKKVCQGTSNKLTQLGTFEDHFLSLQRMFNNCEVVLGNLEITYVQRNYDLSFLKTIQEVAGYVLIALNTVERIPLENLQIIRGNMYYENSYALAVLSNYDANKTGLKELPMRNLQEILHGAVRFSNNPALCNVESIQWRDIVSSDFLSNMSMDFQNHLGSCQKCDPSCPNGSCWGAGEENCQKLTKIICAQQCSGRCRGKSPSDCCHNQCAAGCTGPRESDCLVCRKFRDEATCKDTCPPLMLYNPTTYQMDVNPEGKYSFGATCVKKCPRNYVVTDHGSCVRACGADSYEMEEDGVRKCKKCEGPCRKVCNGIGIGEFKDSLSINATNIKHFKNCTSISGDLHILPVAFRGDSFTHTPPLDPQELDILKTVKEITGFLLIQAWPENRTDLHAFENLEIIRGRTKQHGQFSLAVVSLNITSLGLRSLKEISDGDVAISGNKNLCYANTINWKKLFGTSGQKTKIISNRGENSCKATGQVCHALCSPEGCWGPEPRDCVSCRNVSRGRECVDKCNLLEGEPREFVENSECIQCHPECLPQAMNITCTGRGPDNCIQCAHYIDGPHCVKTCPAGVMGENNTLVWKYADAGHVCHLCHPNCTYGCTGPGLEGCPTNGPKIPSAAASPPCKCPAPNLLGGPSVFIFPPKIKDVLMISLSPIVTCVVVDVSEDDPDVQISWFVNNVEVHTAQTQTHREDYNSTLRVVSALPIQHQDWMSGKEFKCKVNNKDLPAPIERTISKPKGSVRAPQVYVLPPPEEEMTKKQVTLTCMVTDFMPEDIYVEWTNNGKTELNYKNTEPVLDSDGSYFMYSKLRVEKKNWVERNSYSCSVVHEGLHNHHTTKSFSRTPGK

SEQ ID NO: 38 - protein, 854 aa, synthetic construct
DAAQPALEEKKVCQGTSNKLTQLGTFEDHFLSLQRMFNNCEVVLGNLEITYVQRNYDLSFLKTIQEVAGYVLIALNTVERIPLENLQIIRGNMYYENSYALAVLSNYDANKTGLKELPMRNLQEILHGAVRFSNNPALCNVESIQWRDIVSSDFLSNMSMDFQNHLGSCQKCDPSCPNGSCWGAGEENCQKLTKIICAQQCSGRCRGKSPSDCCHNQCAAGCTGPRESDCLVCRKFRDEATCKDTCPPLMLYNPTTYQMDVNPEGKYSFGATCVKKCPRNYVVTDHGSCVRACGADSYEMEEDGVRKCKKCEGPCRKVCNGIGIGEFKDSLSINATNIKHFKNCTSISGDLHILPVAFRGDSFTHTPPLDPQELDILKTVKEITGFLLIQAWPENRTDLHAFENLEIIRGRTKQHGQASLAVVSLNITSLGLRSLKEISDGDVAISGNKNLCYANTINWKKLFGTSGQKTKIISNRGENSCKATGQVCHALCSPEGCWGPEPRDCVSCRNVSRGRECVDKCNLLEGEPREFVENSECIQCHPECLPQAMNITCTGRGPDNCIQCAHYIDGPHCVKTCPAGVMGENNTLVWKYADAGHVCHLCHPNCTYGCTGPGLEGCPTNGPKIPSAAASPPCKCPAPNLLGGPSVFIFPPKIKDVLMISLSPIVTCVVVDVSEDDPDVQISWFVNNVEVHTAQTQTHREDYNSTLRVVSALPIQHQDWMSGKEFKCKVNNKDLPAPIERTISKPKGSVRAPQVYVLPPPEEEMTKKQVTLTCMVTDFMPEDIYVEWTNNGKTELNYKNTEPVLDSDGSYFMYSKLRVEKKNWVERNSYSCSVVHEGLHNHHTTKSFSRTPGK

SEQ ID NO: 39 - protein, 854 aa, synthetic construct
DAAQPALEEKKVCQGTSNKLTQLGTFEDHFLSLQRMFNNCEVVLGNLEITYVQRNYDLSFLKTIQEVAGYVLIALNTVERIPLENLQIIRGNMYYENSYALAVLSNYDANKTGLKELPMRNLQEILHGAVRFSNNPALCNVESIQWRDIVSSDFLSNMSMDFQNHLGSCQKCDPSCPNGSCWGAGEENCQKLTKIICAQQCSGRCRGKSPSDCCHNQCAAGCTGPRESDCLVCRKFRDEATCKDTCPPLMLYNPTTYQMDVNPEGKYSFGATCVKKCPRNYVVTDHGSCVRACGADSYEMEEDGVRKCKKCEGPCRKVCNGIGIGEFKDSLSINATNIKHFKNCTSISGDLHILPVAFRGDSATHTPPLDPQELDILKTVKEITGFLLIQAWPENRTDLHAFENLEIIRGRTKQHGQFSLAVVSLNITSLGLRSLKEISDGDVIISGNKNLCYANTINWKKLFGTSGQKTKIISNRGENSCKATGQVCHALCSPEGCWGPEPRDCVSCRNVSRGRECVDKCNLLEGEPREFVENSECIQCHPECLPQAMNITCTGRGPDNCIQCAHYIDGPHCVKTCPAGVMGENNTLVWKYADAGHVCHLCHPNCTYGCTGPGLEGCPTNGPKIPSAAASPPCKCPAPNLLGGPSVFIFPPKIKDVLMISLSPIVTCVVVDVSEDDPDVQISWFVNNVEVHTAQTQTHREDYNSTLRVVSALPIQHQDWMSGKEFKCKVNNKDLPAPIERTISKPKGSVRAPQVYVLPPPEEEMTKKQVTLTCMVTDFMPEDIYVEWTNNGKTELNYKNTEPVLDSDGSYFMYSKLRVEKKNWVERNSYSCSVVHEGLHNHHTTKSFSRTPGK

SEQ ID NO: 40 - protein, 854 aa, synthetic construct
DAAQPALEEKKVCQGTSNKLTQLGTFEDHFLSLQRMFNNCEVVLGNLEITYVQRNYDLSFLKTIQEVAGYVLIALNTVERIPLENLQIIRGNMYYENSYALAVLSNYDANKTGLKELPMRNLQEILHGAVRFSNNPALCNVESIQWRDIVSSDFLSNMSMDFQNHLGSCQKCDPSCPNGSCWGAGEENCQKLTKIICAQQCSGRCRGKSPSDCCHNQCAAGCTGPRESDCLVCRKFRDEATCKDTCPPLMLYNPTTYQMDVNPEGKYSFGATCVKKCPRNYVVTDHGSCVRACGADSYEMEEDGVRKCKKCEGPCRKVCNGIGIGEFKDSLSINATNIKHFKNCTSISGDLHILPVAFRGDSFTATPPLDPQELDILKTVKEITGFLLIQAWPENRTDLHAFENLEIIRGRTKQHGQFSLAVVSLNITSLGLRSLKEISDGDVIISGNKNLCYANTINWKKLFGTSGQKTKIISNRGENSCKATGQVCHALCSPEGCWGPEPRDCVSCRNVSRGRECVDKCNLLEGEPREFVENSECIQCHPECLPQAMNITCTGRGPDNCIQCAHYIDGPHCVKTCPAGVMGENNTLVWKYADAGHVCHLCHPNCTYGCTGPGLEGCPTNGPKIPSAAASPPCKCPAPNLLGGPSVFIFPPKIKDVLMISLSPIVTCVVVDVSEDDPDVQISWFVNNVEVHTAQTQTHREDYNSTLRVVSALPIQHQDWMSGKEFKCKVNNKDLPAPIERTISKPKGSVRAPQVYVLPPPEEEMTKKQVTLTCMVTDFMPEDIYVEWTNNGKTELNYKNTEPVLDSDGSYFMYSKLRVEKKNWVERNSYSCSVVHEGLHNHHTTKSFSRTPGK

SEQ ID NO: 41 - protein, 854 aa, synthetic construct
DAAQPALEEKKVCQGTSNKLTQLGTFEDHFLSLQRMFNNCEVVLGNLEITYVQRNYDLSFLKTIQEVAGYVLIALNTVERIPLENLQIIRGNMYYENSYALAVLSNYDANKTGLKELPMRNLQEILHGAVRFSNNPALCNVESIQWRDIVSSDFLSNMSMDFQNHLGSCQKCDPSCPNGSCWGAGEENCQKLTKIICAQQCSGRCRGKSPSDCCHNQCAAGCTGPRESDCLVCRKFRDEATCKDTCPPLMLYNPTTYQMDVNPEGKYSFGATCVKKCPRNYVVTDHGSCVRACGADSYEMEEDGVRKCKKCEGPCRKVCNGIGIGEFKDSLSINATNIKHFKNCTSISGDLHILPVAFRGDSATATPPLDPQELDILKTVKEITGFLLIQAWPENRTDLHAFENLEIIRGRTKQHGQFSLAVVSLNITSLGLRSLKEISDGDVIISGNKNLCYANTINWKKLFGTSGQKTKIISNRGENSCKATGQVCHALCSPEGCWGPEPRDCVSCRNVSRGRECVDKCNLLEGEPREFVENSECIQCHPECLPQAMNITCTGRGPDNCIQCAHYIDGPHCVKTCPAGVMGENNTLVWKYADAGHVCHLCHPNCTYGCTGPGLEGCPTNGPKIPSAAASPPCKCPAPNLLGGPSVFIFPPKIKDVLMISLSPIVTCVVVDVSEDDPDVQISWFVNNVEVHTAQTQTHREDYNSTLRVVSALPIQHQDWMSGKEFKCKVNNKDLPAPIERTISKPKGSVRAPQVYVLPPPEEEMTKKQVTLTCMVTDFMPEDIYVEWTNNGKTELNYKNTEPVLDSDGSYFMYSKLRVEKKNWVERNSYSCSVVHEGLHNHHTTKSFSRTPGK

SEQ ID NO: 42 - protein, 854 aa, synthetic construct
DAAQPALEEKKVCQGTSNKLTQLGTFEDHFLSLQRMFNNCEVVLGNLEITYVQRNYDLSFLKTIQEVAGYVLIALNTVERIPLENLQIIRGNMYYENSYALAVLSNYDANKTGLKELPMRNLQEILHGAVRFSNNPALCNVESIQWRDIVSSDFLSNMSMDFQNHLGSCQKCDPSCPNGSCWGAGEENCQKLTKIICAQQCSGRCRGKSPSDCCHNQCAAGCTGPRESDCLVCRKFRDEATCKDTCPPLMLYNPTTYQMDVNPEGKYSFGATCVKKCPRNYVVTDHGSCVRACGADSYEMEEDGVRKCKKCEGPCRKVCNGIGIGEFKDSLSINATNIKHFKNCTSISGDLHILPVAFRGDSFTHTPPLDPQELDILKTVKEITGFLLIQAWPENRTDLHAFENLEIIRGRTKQHGQFSLAVVSLNITSLGLRSLKEISDGDVIISGNKNLCYANTINWKKLFGTAGQKTKIISNRGENSCKATGQVCHALCSPEGCWGPEPRDCVSCRNVSRGRECVDKCNLLEGEPREFVENSECIQCHPECLPQAMNITCTGRGPDNCIQCAHYIDGPHCVKTCPAGVMGENNTLVWKYADAGHVCHLCHPNCTYGCTGPGLEGCPTNGPKIPSAAASPPCKCPAPNLLGGPSVFIFPPKIKDVLMISLSPIVTCVVVDVSEDDPDVQISWFVNNVEVHTAQTQTHREDYNSTLRVVSALPIQHQDWMSGKEFKCKVNNKDLPAPIERTISKPKGSVRAPQVYVLPPPEEEMTKKQVTLTCMVTDFMPEDIYVEWTNNGKTELNYKNTEPVLDSDGSYFMYSKLRVEKKNWVERNSYSCSVVHEGLHNHHTTKSFSRTPGK

SEQ ID NO: 43 - protein, 854 aa, synthetic construct
DAAQPALEEKKVCQGTSNKLTQLGTFEDHFLSLQRMFNNCEVVLGNLEITYVQRNYDLSFLKTIQEVAGYVLIALNTVERIPLENLQIIRGNMYYENSYALAVLSNYDANKTGLKELPMRNLQEILHGAVRFSNNPALCNVESIQWRDIVSSDFLSNMSMDFQNHLGSCQKCDPSCPNGSCWGAGEENCQKLTKIICAQQCSGRCRGKSPSDCCHNQCAAGCTGPRESDCLVCRKFRDEATCKDTCPPLMLYNPTTYQMDVNPEGKYSFGATCVKKCPRNYVVTDHGSCVRACGADSYEMEEDGVRKCKKCEGPCRKVCNGIGIGEFKDSLSINATNIKHFKNCTSISGDLHILPVAFRGDSFTHTPPLDPQELDILKTVKEITGFLLIQAWPENRTDLHAFENLEIIRGRTKQHGQFSLAVVSLNITSLGLRSLKEISDGDVIISGNKNLCYANTINWKKLFGTSGQATKIISNRGENSCKATGQVCHALCSPEGCWGPEPRDCVSCRNVSRGRECVDKCNLLEGEPREFVENSECIQCHPECLPQAMNITCTGRGPDNCIQCAHYIDGPHCVKTCPAGVMGENNTLVWKYADAGHVCHLCHPNCTYGCTGPGLEGCPTNGPKIPSAAASPPCKCPAPNLLGGPSVFIFPPKIKDVLMISLSPIVTCVVVDVSEDDPDVQISWFVNNVEVHTAQTQTHREDYNSTLRVVSALPIQHQDWMSGKEFKCKVNNKDLPAPIERTISKPKGSVRAPQVYVLPPPEEEMTKKQVTLTCMVTDFMPEDIYVEWTNNGKTELNYKNTEPVLDSDGSYFMYSKLRVEKKNWVERNSYSCSVVHEGLHNHHTTKSFSRTPGK

SEQ ID NO: 44 - protein, 854 aa, synthetic construct
DAAQPALEEKKVCQGTSNKLTQLGTFEDHFLSLQRMFNNCEVVLGNLEITYVQRNYDLSFLKTIQEVAGYVLIALNTVERIPLENLQIIRGNMYYENSYALAVLSNYDANKTGLKELPMRNLQEILHGAVRFSNNPALCNVESIQWRDIVSSDFLSNMSMDFQNHLGSCQKCDPSCPNGSCWGAGEENCQKLTKIICAQQCSGRCRGKSPSDCCHNQCAAGCTGPRESDCLVCRKFRDEATCKDTCPPLMLYNPTTYQMDVNPEGKYSFGATCVKKCPRNYVVTDHGSCVRACGADSYEMEEDGVRKCKKCEGPCRKVCNGIGIGEFKDSLSINATNIKHFKNCTSISGDLHILPVAFRGDSFTHTPPLDPQELDILKTVKEITGFLLIQAWPENRTDLHAFENLEIIRGRTKQHGQFSLAVDSLNITSLGLRSLKEISDGDVIISGNKNLCYANTINWKKLFGTSGQKTKIISNRGENSCKATGQVCHALCSPEGCWGPEPRDCVSCRNVSRGRECVDKCNLLEGEPREFVENSECIQCHPECLPQAMNITCTGRGPDNCIQCAHYIDGPHCVKTCPAGVMGENNTLVWKYADAGHVCHLCHPNCTYGCTGPGLEGCPTNGPKIPSAAASPPCKCPAPNLLGGPSVFIFPPKIKDVLMISLSPIVTCVVVDVSEDDPDVQISWFVNNVEVHTAQTQTHREDYNSTLRVVSALPIQHQDWMSGKEFKCKVNNKDLPAPIERTISKPKGSVRAPQVYVLPPPEEEMTKKQVTLTCMVTDFMPEDIYVEWTNNGKTELNYKNTEPVLDSDGSYFMYSKLRVEKKNWVERNSYSCSVVHEGLHNHHTTKSFSRTPGK

SEQ ID NO: 45 - protein, 854 aa, synthetic construct
DAAQPALEEKKVCQGTSNKLTQLGTFEDHFLSLQRMFNNCEVVLGNLEITYVQRNYDLSFLKTIQEVAGYVLIALNTVERIPLENLQIIRGNMYYENSYALAVLSNYDANKTGLKELPMRNLQEILHGAVRFSNNPALCNVESIQWRDIVSSDFLSNMSMDFQNHLGSCQKCDPSCPNGSCWGAGEENCQKLTKIICAQQCSGRCRGKSPSDCCHNQCAAGCTGPRESDCLVCRKFRDEATCKDTCPPLMLYNPTTYQMDVNPEGKYSFGATCVKKCPRNYVVTDHGSCVRACGADSYEMEEDGVRKCKKCEGPCRKVCNGIGIGEFKDSLSINATNIKHFKNCTSISGDLHILPVAFRGDSFTHTPPLDPQELDILKTVKEITGFLLIQAWPENRTDLHAFENLEIIRGRTKQHGQFSLAVGSLNITSLGLRSLKEISDGDVIISGNKNLCYANTINWKKLFGTSGQKTKIISNRGENSCKATGQVCHALCSPEGCWGPEPRDCVSCRNVSRGRECVDKCNLLEGEPREFVENSECIQCHPECLPQAMNITCTGRGPDNCIQCAHYIDGPHCVKTCPAGVMGENNTLVWKYADAGHVCHLCHPNCTYGCTGPGLEGCPTNGPKIPSAAASPPCKCPAPNLLGGPSVFIFPPKIKDVLMISLSPIVTCVVVDVSEDDPDVQISWFVNNVEVHTAQTQTHREDYNSTLRVVSALPIQHQDWMSGKEFKCKVNNKDLPAPIERTISKPKGSVRAPQVYVLPPPEEEMTKKQVTLTCMVTDFMPEDIYVEWTNNGKTELNYKNTEPVLDSDGSYFMYSKLRVEKKNWVERNSYSCSVVHEGLHNHHTTKSFSRTPGK

SEQ ID NO: 46 - protein, 854 aa, synthetic construct
DAAQPALEEKKVCQGTSNKLTQLGTFEDHFLSLQRMFNNCEVVLGNLEITYVQRNYDLSFLKTIQEVAGYVLIALNTVERIPLENLQIIRGNMYYENSYALAVLSNYDANKTGLKELPMRNLQEILHGAVRFSNNPALCNVESIQWRDIVSSDFLSNMSMDFQNHLGSCQKCDPSCPNGSCWGAGEENCQKLTKIICAQQCSGRCRGKSPSDCCHNQCAAGCTGPRESDCLVCRKFRDEATCKDTCPPLMLYNPTTYQMDVNPEGKYSFGATCVKKCPRNYVVTDHGSCVRACGADSYEMEEDGVRKCKKCEGPCRKVCNGIGIGEFKDSLSINATNIKHFKNCTSISGDLHILPVAFRGDSFTHTPPLDPQELDILKTVKEITGFLLIQAWPENRTDLHAFENLEIIRGRTKQHGQFSLAVVRLNITSLGLRSLKEISDGDVIISGNKNLCYANTINWKKLFGTSGQKTKIISNRGENSCKATGQVCHALCSPEGCWGPEPRDCVSCRNVSRGRECVDKCNLLEGEPREFVENSECIQCHPECLPQAMNITCTGRGPDNCIQCAHYIDGPHCVKTCPAGVMGENNTLVWKYADAGHVCHLCHPNCTYGCTGPGLEGCPTNGPKIPSAAASPPCKCPAPNLLGGPSVFIFPPKIKDVLMISLSPIVTCVVVDVSEDDPDVQISWFVNNVEVHTAQTQTHREDYNSTLRVVSALPIQHQDWMSGKEFKCKVNNKDLPAPIERTISKPKGSVRAPQVYVLPPPEEEMTKKQVTLTCMVTDFMPEDIYVEWTNNGKTELNYKNTEPVLDSDGSYFMYSKLRVEKKNWVERNSYSCSVVHEGLHNHHTTKSFSRTPGK

SEQ ID NO: 47 - protein, 854 aa, synthetic construct
DAAQPALEEKKVCQGTSNKLTQLGTFEDHFLSLQRMFNNCEVVLGNLEITYVQRNYDLSFLKTIQEVAGYVLIALNTVERIPLENLQIIRGNMYYENSYALAVLSNYDANKTGLKELPMRNLQEILHGAVRFSNNPALCNVESIQWRDIVSSDFLSNMSMDFQNHLGSCQKCDPSCPNGSCWGAGEENCQKLTKIICAQQCSGRCRGKSPSDCCHNQCAAGCTGPRESDCLVCRKFRDEATCKDTCPPLMLYNPTTYQMDVNPEGKYSFGATCVKKCPRNYVVTDHGSCVRACGADSYEMEEDGVRKCKKCEGPCRKVCNGIGIGEFKDSLSINATNIKHFKNCTSISGDLHILPVAFRGDSFTHTPPLDPQELDILKTVKEITGFLLIQAWPENRTDLHAFENLEIIRGRTKQHGQFSLAVVSLNITSLGLRSLKEISDGDVIILGNKNLCYANTINWKKLFGTSGQKTKIISNRGENSCKATGQVCHALCSPEGCWGPEPRDCVSCRNVSRGRECVDKCNLLEGEPREFVENSECIQCHPECLPQAMNITCTGRGPDNCIQCAHYIDGPHCVKTCPAGVMGENNTLVWKYADAGHVCHLCHPNCTYGCTGPGLEGCPTNGPKIPSAAASPPCKCPAPNLLGGPSVFIFPPKIKDVLMISLSPIVTCVVVDVSEDDPDVQISWFVNNVEVHTAQTQTHREDYNSTLRVVSALPIQHQDWMSGKEFKCKVNNKDLPAPIERTISKPKGSVRAPQVYVLPPPEEEMTKKQVTLTCMVTDFMPEDIYVEWTNNGKTELNYKNTEPVLDSDGSYFMYSKLRVEKKNWVERNSYSCSVVHEGLHNHHTTKSFSRTPGK

SEQ ID NO: 48 - protein, 854 aa, synthetic construct
DAAQPALEEKKVCQGTSNKLTQLGTFEDHFLSLQRMFNNCEVVLGNLEITYVQRNYDLSFLKTIQEVAGYVLIALNTVERIPLENLQIIRGNMYYENSYALAVLSNYDANKTGLKELPMRNLQEILHGAVRFSNNPALCNVESIQWRDIVSSDFLSNMSMDFQNHLGSCQKCDPSCPNGSCWGAGEENCQKLTKIICAQQCSGRCRGKSPSDCCHNQCAAGCTGPRESDCLVCRKFRDEATCKDTCPPLMLYNPTTYQMDVNPEGKYSFGATCVKKCPRNYVVTDHGSCVRACGADSYEMEEDGVRKCKKCEGPCRKVCNGIGIGEFKDSLSINATNIKHFKNCTSISGDLHILPVAFRGDSFTHTPPLDPQELDILKTVKEITGFLLIQAWPENRTDLHAFENLEIIRGRTKQHGQFSLAVVSLNITSLGLRSLKEISDGDVIISRNKNLCYANTINWKKLFGTSGQKTKIISNRGENSCKATGQVCHALCSPEGCWGPEPRDCVSCRNVSRGRECVDKCNLLEGEPREFVENSECIQCHPECLPQAMNITCTGRGPDNCIQCAHYIDGPHCVKTCPAGVMGENNTLVWKYADAGHVCHLCHPNCTYGCTGPGLEGCPTNGPKIPSAAASPPCKCPAPNLLGGPSVFIFPPKIKDVLMISLSPIVTCVVVDVSEDDPDVQISWFVNNVEVHTAQTQTHREDYNSTLRVVSALPIQHQDWMSGKEFKCKVNNKDLPAPIERTISKPKGSVRAPQVYVLPPPEEEMTKKQVTLTCMVTDFMPEDIYVEWTNNGKTELNYKNTEPVLDSDGSYFMYSKLRVEKKNWVERNSYSCSVVHEGLHNHHTTKSFSRTPGK

SEQ ID NO: 49 - protein, 854 aa, synthetic construct
DAAQPALEEKKVCQGTSNKLTQLGTFEDHFLSLQRMFNNCEVVLGNLEITYVQRNYDLSFLKTIQEVAGYVLIALNTVERIPLENLQIIRGNMYYENSYALAVLSNYDANKTGLKELPMRNLQEILHGAVRFSNNPALCNVESIQWRDIVSSDFLSNMSMDFQNHLGSCQKCDPSCPNGSCWGAGEENCQKLTKIICAQQCSGRCRGKSPSDCCHNQCAAGCTGPRESDCLVCRKFRDEATCKDTCPPLMLYNPTTYQMDVNPEGKYSFGATCVKKCPRNYVVTDHGSCVRACGADSYEMEEDGVRKCKKCEGPCRKVCNGIGIGEFKDSLSINATNIKHFKNCTSISGDLHILPVAFRGDSFTHTPPLDPQELDILKTVKEITGFLLIQAWPENRTDLHAFENLEIIRGRTKQHGQFSLAVVSLNITSLGLRSLKEISDGDVIISGNKNLCYANTINWKKLFGTSGQKTEIISNRGENSCKATGQVCHALCSPEGCWGPEPRDCVSCRNVSRGRECVDKCNLLEGEPREFVENSECIQCHPECLPQAMNITCTGRGPDNCIQCAHYIDGPHCVKTCPAGVMGENNTLVWKYADAGHVCHLCHPNCTYGCTGPGLEGCPTNGPKIPSAAASPPCKCPAPNLLGGPSVFIFPPKIKDVLMISLSPIVTCVVVDVSEDDPDVQISWFVNNVEVHTAQTQTHREDYNSTLRVVSALPIQHQDWMSGKEFKCKVNNKDLPAPIERTISKPKGSVRAPQVYVLPPPEEEMTKKQVTLTCMVTDFMPEDIYVEWTNNGKTELNYKNTEPVLDSDGSYFMYSKLRVEKKNWVERNSYSCSVVHEGLHNHHTTKSFSRTPGK

SEQ ID NO: 50 - protein, 854 aa, synthetic construct
DAAQPALEEKKVCQGTSNKLTQLGTFEDHFLSLQRMFNNCEVVLGNLEITYVQRNYDLSFLKTIQEVAGYVLIALNTVERIPLENLQIIRGNMYYENSYALAVLSNYDANKTGLKELPMRNLQEILHGAVRFSNNPALCNVESIQWRDIVSSDFLSNMSMDFQNHLGSCQKCDPSCPNGSCWGAGEENCQKLTKIICAQQCSGRCRGKSPSDCCHNQCAAGCTGPRESDCLVCRKFRDEATCKDTCPPLMLYNPTTYQMDVNPEGKYSFGATCVKKCPRNYVVTDHGSCVRACGADSYEMEEDGVRKCKKCEGPCRKVCNGIGIGEFKDSLSINATNIKHFKNCTSISGDLHILPVAFRGDSFTHTPPLDPQELDILKTVKEITGFLLIQAWPENRTDLHAFENLEIIRGRTKQHGQFSLAVVSLNITSLGLRSLKEISDGDVIISGNKNLCYANTINWKKLFGTSGQKTKIIRNRGENSCKATGQVCHALCSPEGCWGPEPRDCVSCRNVSRGRECVDKCNLLEGEPREFVENSECIQCHPECLPQAMNITCTGRGPDNCIQCAHYIDGPHCVKTCPAGVMGENNTLVWKYADAGHVCHLCHPNCTYGCTGPGLEGCPTNGPKIPSAAASPPCKCPAPNLLGGPSVFIFPPKIKDVLMISLSPIVTCVVVDVSEDDPDVQISWFVNNVEVHTAQTQTHREDYNSTLRVVSALPIQHQDWMSGKEFKCKVNNKDLPAPIERTISKPKGSVRAPQVYVLPPPEEEMTKKQVTLTCMVTDFMPEDIYVEWTNNGKTELNYKNTEPVLDSDGSYFMYSKLRVEKKNWVERNSYSCSVVHEGLHNHHTTKSFSRTPGK

SEQ ID NO: 51 - protein, 653 aa, synthetic construct
MRPSGTARTTLLVLLTALCAAGGALEEKKVCQGTSNRLTQLGTFEDHFLSLQRMYNNCEVVLGNLEITYVQRNYDLSFLKTIQEVAGYVLIALNTVERIPLENLQIIRGNALYENTYALAILSNYGTNRTGLRELPMRNLQEILIGAVRFSNNPILCNMDTIQWRDIVQNVFMSNMSMDLQSHPSSCPKCDPSCPNGSCWGGGEENCQKLTKIICAQQCSHRCRGRSPSDCCHNQCAAGCTGPRESDCLVCQKFQDEATCKDTCPPLMLYNPTTYQMDVNPEGKYSFGATCVKKCPRNYVVTDHGSCVRACGPDYYEVEEDGIRKCKKCDGPCRKVCNGIGIGEFKDTLSINATNIKHFKYCTAISGDLHILPVAFKGDSFTRTPPLDPRELEILKTVKEITGFLLIQAWPDNWTDLHAFENLEIIRGRTKQHGQFSLAVVGLNITSLGLRSLKEISDGDVIISGNRNLCYANTINWKKLFGTPNQKTKIMNNRAEKDCKAVNHVCNPLCSSEGCWGPEPRDCVSCQNVSRGRECVEKCNILEGEPREFVENSECIQCHPECLPQAMNITCTGRGPDNCIQCAHYIDGPHCVKTCPAGIMGENNTLVWKYADANNVCHLCHANCTYGCAGPGLQGCEVWPSGPKIPSHHHHHH

SEQ ID NO: 52 - protein, 651 aa, synthetic construct
MRPSGTAGAALLALLAALCPASRALEEKKVCQGTSNKLTQLGTFEDHFLSLQRMFNNCEVVLGNLEITYVQRNYDLSFLKTIQEVAGYVLIALNTVERIPLENLQIIRGNMYYENSYALAVLSNYDANKTGLKELPMRNLQEILHGAVRFSNNPALCNVESIQWRDIVSSEFLSNMSMDFQNHLGSCQKCDPSCPNGSCWGAGEENCQKLTKIICAQQCSGRCRGKSPSDCCHNQCAAGCTGPRESDCLVCRKFRDEATCKDTCPPLMLYNPTTYQMDVNPEGKYSFGATCVKKCPRNYVVTDHGSCVRACGADSYEMEEDGVRKCKKCEGPCRKVCNGIGIGEFKDTLSINATNIKHFKNCTSISGDLHILPVAFRGDSFTHTPPLDPQELDILKTVKEITGFLLIQAWPENRTDLHAFENLEIIRGRTKQHGQFSLAVVSLNITSLGLRSLKEISDGDVIISGNKNLCYANTINWKKLFGTSSQKTKIISNRGENSCKATGQVCHALCSPEGCWGPEPRDCVSCQNVSRGRECVDKCNILEGEPREFVENSECIQCHPECLPQVMNITCTGRGPDNCIQCAHYIDGPHCVKTCPAGVMGENNTLVWKYADAGHVCHLCHPNCTYGCTGPGLEGCARNGPKIPSHHHHHH

SEQ ID NO: 53 - protein, 636 aa, synthetic construct
DAAQPALEEKKVCQGTSNKLTQLGTFEDHFLSLQRMFNNCEVVLGNLEITYVQRNYDLSFLKTIQEVAGYVLIALNTVERIPLENLQIIRGNMYYENSYALAVLSNYDANKTGLKELPMRNLQEILHGAVRFSNNPALCNVESIQWRDIVSSDFLSNMSMDFQNHLGSCQKCDPSCPNGSCWGAGEENCQKLTKIICAQQCSGRCRGKSPSDCCHNQCAAGCTGPRESDCLVCRKFRDEATCKDTCPPLMLYNPTTYQMDVNPEGKYSFGATCVKKCPRNYVVTDHGSCVRACGADSYEMEEDGVRKCKKCEGPCRKVCNGIGIGEFKDSLSINATNIKHFKNCTSISGDLHILPVAFRGDSFTHTPPLDPQELDILKTVKEITGFLLIQAWPENRTDLHAFENLEIIRGRTKQHGQFSLAVVSLNITSLGLRSLKEISDGDVIISGNKNLCYANTINWKKLFGTSGQKTKIISNRGENSCKATGQVCHALCSPEGCWGPEPRDCVSCRNVSRGRECVDKCNLLEGEPREFVENSECIQCHPECLPQAMNITCTGRGPDNCIQCAHYIDGPHCVKTCPAGVMGENNTLVWKYADAGHVCHLCHPNCTYGCTGPGLEGCPTNGPKIPSAAAHHHHHH

SEQ ID NO: 54 - protein, 1210 aa, synthetic construct [sequence omitted]

SEQ ID NO: 55 - protein, 1210 aa, synthetic construct
MRPSGTAGAALLALLAALCPASRALEEKKVCQGTSNKLTQLGTFEDHFLSLQRMFNNCEVVLGNLEITYVQRNYDLSFLKTIQEVAGYVLIALNTVERIPLENLQIIRGNMYYENSYALAVLSNYDANKTGLKELPMRNLQEILHGAVRFSNNPALCNVESIQWRDIVSSDFLSNMSMDFQNHLGSCQKCDPSCPNGSCWGAGEENCQKLTKIICAQQCSGRCRGKSPSDCCHNQCAAGCTGPRESDCLVCRKFRDEATCKDTCPPLMLYNPTTYQMDVNPEGKYSFGATCVKKCPRNYVVTDHGSCVRACGADSYEMEEDGVRKCKKCEGPCRKVCNGIGIGEFKDSLSINATNIKHFKNCTSISGDLHILPVAFRGDSFTHTPPLDPQELDILKTVKEITGFLLIQAWPENRTDLHAFENLEIIRGRTKQHGQFSLAVVSLNITSLGLRSLKEISDGDVIISRNKNLCYANTINWKKLFGTSGQKTKIISNRGENSCKATGQVCHALCSPEGCWGPEPRDCVSCRNVSRGRECVDKCNLLEGEPREFVENSECIQCHPECLPQAMNITCTGRGPDNCIQCAHYIDGPHCVKTCPAGVMGENNTLVWKYADAGHVCHLCHPNCTYGCTGPGLEGCPTNGPKIPSIATGMVGALLLLLVVALGIGLFMRRRHIVRKRTLRRLLQERELVEPLTPSGEAPNQALLRILKETEFKKIKVLGSGAFGTVYKGLWIPEGEKVKIPVAIKELREATSPKANKEILDEAYVMASVDNPHVCRLLGICLTSTVQLITQLMPFGCLLDYVREHKDNIGSQYLLNWCVQIAKGMNYLEDRRLVHRDLAARNVLVKTPQHVKITDFGLAKLLGAEEKEYHAEGGKVPIKWMALESILHRIYTHQSDVWSYGVTVWELMTFGSKPYDGIPASEISSILEKGERLPQPPICTIDVYMIMVKCWMIDADSRPKFRELIIEFSKMARDPQRYLVIQGDERMHLPSPTDSNFYRALMDEEDMDDVVDADEYLIPQQGFFSSPSTSRTPLLSSLSATSNNSTVACIDRNGLQSCPIKEDSFLQRYSSDPTGALTEDSIDDTFLPVPEYINQSVPKRPAGSVQNPVYHNQPLNPAPSRDPHYQDPHSTAVGNPEYLNTVQPTCVNSTFDSPAHWAQKGSHQISLDNPDYQQDFFPKEAKPNGIFKGSTAENAEYLRVAPQSSEFIGA

SEQ ID NO: 56 - protein, 1210 aa, synthetic construct
MRPSGTAGAALLALLAALCPASRALEEKKVCQGTSNKLTQLGTFEDHFLSLQRMFNNCEVVLGNLEITYVQRNYDLSFLKTIQEVAGYVLIALNTVERIPLENLQIIRGNMYYENSYALAVLSNYDANKTGLKELPMRNLQEILHGAVRFSNNPALCNVESIQWRDIVSSDFLSNMSMDFQNHLGSCQKCDPSCPNGSCWGAGEENCQKLTKIICAQQCSGRCRGKSPSDCCHNQCAAGCTGPRESDCLVCRKFRDEATCKDTCPPLMLYNPTTYQMDVNPEGKYSFGATCVKKCPRNYVVTDHGSCVRACGADSYEMEEDGVRKCKKCEGPCRKVCNGIGIGEFKDSLSINATNIKHFKNCTSISGDLHILPVAFRGDSFTHTPPLDPQELDILKTVKEITGFLLIQAWPENRTDLHAFENLEIIRGRTKQHGQFSLAVVSLNITSLGLRSLKEISDGDVIISGNKNLCYANTINWKKLFGTSGQKTKIIRNRGENSCKATGQVCHALCSPEGCWGPEPRDCVSCRNVSRGRECVDKCNLLEGEPREFVENSECIQCHPECLPQAMNITCTGRGPDNCIQCAHYIDGPHCVKTCPAGVMGENNTLVWKYADAGHVCHLCHPNCTYGCTGPGLEGCPTNGPKIPSIATGMVGALLLLLVVALGIGLFMRRRHIVRKRTLRRLLQERELVEPLTPSGEAPNQALLRILKETEFKKIKVLGSGAFGTVYKGLWIPEGEKVKIPVAIKELREATSPKANKEILDEAYVMASVDNPHVCRLLGICLTSTVQLITQLMPFGCLLDYVREHKDNIGSQYLLNWCVQIAKGMNYLEDRRLVHRDLAARNVLVKTPQHVKITDFGLAKLLGAEEKEYHAEGGKVPIKWMALESILHRIYTHQSDVWSYGVTVWELMTFGSKPYDGIPASEISSILEKGERLPQPPICTIDVYMIMVKCWMIDADSRPKFRELIIEFSKMARDPQRYLVIQGDERMHLPSPTDSNFYRALMDEEDMDDVVDADEYLIPQQGFFSSPSTSRTPLLSSLSATSNNSTVACIDRNGLQSCPIKEDSFLQRYSSDPTGALTEDSIDDTFLPVPEYINQSVPKRPAGSVQNPVYHNQPLNPAPSRDPHYQDPHSTAVGNPEYLNTVQPTCVNSTFDSPAHWAQKGSHQISLDNPDYQQDFFPKEAKPNGIFKGSTAENAEYLRVAPQSSEFIGA

SEQ ID NO: 57 - protein, 216 aa, synthetic construct
QSVLTQPPSVSGAPGQRVTISCSGGSSNVGRNGVNWFQHLPEKAPKLLIYYDAFLSSGVSDRFSGSKSGTSASLAIRGLQSDDEADYYCAAWDDSLYSWVFGGGTKLTVLGQPKAAPSVTLFPPSSEELQANKATLVCLISDFYPGAVTVAWKADSSPVKAGVETTTPSKQSNNKYAASSYLSLTPEQWKSHRSYSCQVTHEGSTVEKTVAPTECS

SEQ ID NO: 58 - protein, 450 aa, synthetic construct
QVQLVQSGGGVVQPGGSLRLSCAASGFTFSSYGMHWVRQAPGKGLEWVAFIRYDGSNKYYADSVKGRFTISRDNSKNTLYLQMNSLRAEDTAVYYCAKDGNSGYDSMDYWGQGTLVTVSSASTKGPSVFPLAPSSKSTSGGTAALGCLVKDYFPEPVTVSWNSGALTSGVHTFPAVLQSSGLYSLSSVVTVPSSSLGTQTYICNVNHKPSNTKVDKKVEPKSCDKTHTCPPCPAPELLGGPSVFLFPPKPKDTLMISRTPEVTCVVVDVSHEDPEVKFNWYVDGVEVHNAKTKPREEQYNSTYRVVSVLTVLHQDWLNGKEYKCKVSNKALPAPIEKTISKAKGQPREPQVYTLPPSREEMTKNQVSLTCLVKGFYPSDIAVEWESNGQPENNYKTTPPVLDSDGSFFLYSKLTVDKSRWQQGNVFSCSVMHEALHNHYTQKSLSLSPGK

SEQ ID NO: 59 - protein, 741 aa, synthetic construct
MRPSGTAGAALLALLAALCPASRALEEKKVCQGTSNKLTQLGTFEDHFLSLQRMFNNCEVVLGNLEITYVQRNYDLSFLKTIQEVAGYVLIALNTVERIPLENLQIIRGNMYYENSYALAVLSNYDANKTGLKELPMRNLQEILHGAVRFSNNPALCNVESIQWRDIVSSDFLSNMSMDFQNHLGSCQKCDPSCPNGSCWGAGEENCQKLTKIICAQQCSGRCRGKSPSDCCHNQCAAGCTGPRESDCLVCRKFRDEATCKDTCPPLMLYNPTTYQMDVNPEGKYSFGATCVKKCPRNYVVTDHGSCVRACGADSYEMEEDGVRKCKKCEGPCRKVCNGIGIGEFKDSLSINATNIKHFKNCTSISGDLHILPVAFRGDSFTHTPPLDPQELDILKTVKEITGFLLIQAWPENRTDLHAFENLEIIRGRTKQHGQFSLAVVSLNITSLGLRSLKEISDGDVIISGNKNLCYANTINWKKLFGTSGQKTKIISNRGENSCKATGQVCHALCSPEGCWGPEPRDCVSCRNVSRGRECVDKCNLLEGEPREFVENSECIQCHPECLPQAMNITCTGRGPDNCIQCAHYIDGPHCVKTCPAGVMGENNTLVWKYADAGHVCHLCHPNCTYGCTGPGLEGCPTNGPKIPSIATGMVGALLLLLVVALGIGLFMRRRHIVRKRTLAAAGSGGGGSMGVITDSLAVVLQRRDWENPGVTQLNRLAARPPFASWRNSEEARTDRPSQQL

SEQ ID NO: 60 - protein, 1682 aa, synthetic construct
MRPSGTAGAALLALLAALCPASRALEEKKVCQGTSNKLTQLGTFEDHFLSLQRMFNNCEVVLGNLEITYVQRNYDLSFLKTIQEVAGYVLIALNTVERIPLENLQIIRGNMYYENSYALAVLSNYDANKTGLKELPMRNLQEILHGAVRFSNNPALCNVESIQWRDIVSSDFLSNMSMDFQNHLGSCQKCDPSCPNGSCWGAGEENCQKLTKIICAQQCSGRCRGKSPSDCCHNQCAAGCTGPRESDCLVCRKFRDEATCKDTCPPLMLYNPTTYQMDVNPEGKYSFGATCVKKCPRNYVVTDHGSCVRACGADSYEMEEDGVRKCKKCEGPCRKVCNGIGIGEFKDSLSINATNIKHFKNCTSISGDLHILPVAFRGDSFTHTPPLDPQELDILKTVKEITGFLLIQAWPENRTDLHAFENLEIIRGRTKQHGQFSLAVVSLNITSLGLRSLKEISDGDVIISGNKNLCYANTINWKKLFGTSGQKTKIISNRGENSCKATGQVCHALCSPEGCWGPEPRDCVSCRNVSRGRECVDKCNLLEGEPREFVENSECIQCHPECLPQAMNITCTGRGPDNCIQCAHYIDGPHCVKTCPAGVMGENNTLVWKYADAGHVCHLCHPNCTYGCTGPGLEGCPTNGPKIPSIATGMVGALLLLLVVALGIGLFMRRRHIVRKRTLAAAGSGGGGSPPFASWRNSEEARTDRPSQQLRSLNGEWRFAWFPAPEAVPESWLECDLPEADTVVVPSNWQMHGYDAPIYTNVTYPITVNPPFVPTENPTGCYSLTFNVDESWLQEGQTRIIFDGVNSAFHLWCNGRWVGYGQDSRLPSEFDLSAFLRAGENRLAVMVLRWSDGSYLEDQDMWRMSGIFRDVSLLHKPTTQISDFHVATRFNDDFSRAVLEAEVQMCGELRDYLRVTVSLWQGETQVASGTAPFGGEIIDERGGYADRVTLRLNVENPKLWSAEIPNLYRAVVELHTADGTLIEAEACDVGFREVRIENGLLLLNGKPLLIRGVNRHEHHPLHGQVMDEQTMVQDILLMKQNNFNAVRCSHYPNHPLWYTLCDRYGLYVVDEANIETHGMVPMNRLTDDPRWLPAMSERVTRMVQRDRNHPSVIIWSLGNESGHGANHDALYRWIKSVDPSRPVQYEGGGADTTATDIICPMYARVDEDQPFPAVPKWSIKKWLSLPGETRPLILCEYAHAMGNSLGGFAKYWQAFRQYPRLQGGFVWDWVDQSLIKYDENGNPWSAYGGDFGDTPNDRQFCMNGLVFADRTPHPALTEAKHQQQFFQFRLSGQTIEVTSEYLFRHSDNELLHWMVALDGKPLASGEVPLDVAPQGKQLIELPELPQPESAGQLWLTVRVVQPNATAWSEAGHISAWQQWRLAENLSVTLPAASHAIPHLTTSEMDFCIELGNKRWQFNRQSGFLSQMWIGDKKQLLTPLRDQFTRAPLDNDIGVSEATRIDPNAWVERWKAAGHYQAEAALLQCTADTLADAVLITTAHAWQHQGKTLFISRKTYRIDGSGQMAITVDVEVASDTPHPARIGLNCQLAQVAERVNWLGLGPQENYPDRLTAACFDRWDLPLSDMYTPYVFPSENGLRCGTRELNYGPHQWRGDFQFNISRYSQQQLMETSHRHLLHAEEGTWLNIDGFHMGIGGDDSWSPSVSAEFQLSAGRYHYQLVWCQK

SEQ ID NO: 61 - protein, 170 aa, synthetic construct
KVCNGIGIGEFKDSLSINATNIKHFKNCTSISGDLHILPVAFRGDSFTHTPPLDPQELDILKTVKEITGFLLIQAWPENRTDLHAFENLEIIRGRTKQHGQFSLAVVSLNITSLGLRSLKEISDGDVIISGNKNLCYANTINWKKLFGTSGQKTKIISNRGENSCKATGQ

SEQ ID NO: 62 - protein, 238 aa, synthetic construct
QVQLKQSGPGLVQPSQSLSITCTVSGFSLTNYGVHWVRQSPGKGLEWLGVIWSGGNTDYNTPFTSRLSINKDNSKSQVFFKMNSLQSNDTAIYYCARALTYYDYEFAYWGQGTLVTVSAASTKGPSVFPLAPSSKSTSGGTAALGCLVKDYFPEPVTVSWNSGALTSGVHTFPAVLQSSGLYSLSSVVTVPSSSLGTQTYICNVNHKPSNTKVDKKVEPKSCGGSGGGGSGGHHHHHH

SEQ ID NO: 63 - protein, 636 aa, synthetic construct
DAAQPALEEKKVCQGTSNKLTQLGTFEDHFLSLQRMFNNCEVVLGNLEITYVQRNYDLSFLKTIQEVAGYVLIALNTVERIPLENLQIIRGNMYYENSYALAVLSNYDANKTGLKELPMRNLQEILHGAVRFSNNPALCNVESIQWRDIVSSDFLSNMSMDFQNHLGSCQKCDPSCPNGSCWGAGEENCQKLTKIICAQQCSGRCRGKSPSDCCHNQCAAGCTGPRESDCLVCRKFRDEATCKDTCPPLMLYNPTTYQMDVNPEGKYSFGATCVKKCPRNYVVTDHGSCVRACGADSYEMEEDGVRKCKKCEGPCRKVCNGIGIGEFKDSLSINATNIKHFKNCTSISGDLHILPVAFRGDSFTHTPPLDPQELDILKTVKEITGFLLIQAWPENRTDLHAFENLEIIRGRTKQHGPFSLAVVSLNITSLGLRSLKEISDGDVIISGNKNLCYANTINWKKLFGTSGQKTKIISNRGENSCKATGQVCHALCSPEGCWGPEPRDCVSCRNVSRGRECVDKCNLLEGEPREFVENSECIQCHPECLPQAMNITCTGRGPDNCIQCAHYIDGPHCVKTCPAGVMGENNTLVWKYADAGHVCHLCHPNCTYGCTGPGLEGCPTNGPKIPSAAAHHHHHH

SEQ ID NO: 64 - protein, 636 aa, synthetic construct
DAAQPALEEKKVCQGTSNKLTQLGTFEDHFLSLQRMFNNCEVVLGNLEITYVQRNYDLSFLKTIQEVAGYVLIALNTVERIPLENLQIIRGNMYYENSYALAVLSNYDANKTGLKELPMRNLQEILHGAVRFSNNPALCNVESIQWRDIVSSDFLSNMSMDFQNHLGSCQKCDPSCPNGSCWGAGEENCQKLTKIICAQQCSGRCRGKSPSDCCHNQCAAGCTGPRESDCLVCRKFRDEATCKDTCPPLMLYNPTTYQMDVNPEGKYSFGATCVKKCPRNYVVTDHGSCVRACGADSYEMEEDGVRKCKKCEGPCRKVCNGIGIGEFKDSLSINATNIKHFKNCTSISGDLHILPVAFRGDSFTHTPPLDPQELDILKTVKEITGFLLIQAWPENRTDLHAFENLEIIRGRTKQHGQFSLAVDSLNITSLGLRSLKEISDGDVIISGNKNLCYANTINWKKLFGTSGQKTKIISNRGENSCKATGQVCHALCSPEGCWGPEPRDCVSCRNVSRGRECVDKCNLLEGEPREFVENSECIQCHPECLPQAMNITCTGRGPDNCIQCAHYIDGPHCVKTCPAGVMGENNTLVWKYADAGHVCHLCHPNCTYGCTGPGLEGCPTNGPKIPSAAAHHHHHH

SEQ ID NO: 65 - protein, 616 aa, synthetic construct
DAAQPALEEKKVCQGTSNKLTQLGTFEDHFLSLQRMFNNCEVVLGNLEITYVQRNYDLSFLKTIQEVAGYVLIALNTVERIPLENLQIIRGNMYYENSYALAVLSNYDANKTGLKELPMRNLQEILHGAVRFSNNPALCNVESIQWRDIVSSDFLSNMSMDFQNHLGSCQKCDPSCPNGSCWGAGEENCQKLTKIICAQQCSGRCRGKSPSDCCHNQCAAGCTGPRESDCLVCRKFRDEATCKDTCPPLMLYNPTTYQMDVNPEGKYSFGATCVKKCPRNYVVTDHGSCVRACGADSYEMEEDGVRKCKKCEGPCRKVCNGIGIGEFKDSLSINATNIKHFKNCTSISGDLHILPVAFRGDSFTHTPPLDPQELDILKTVKEITGFLLIQAWPENRTDLHAFENLEIIRGRTKQHGQFSLAVVSLNITSLGLRSLKEISDGDVIILGNKNLCYANTINWKKLFGTSGQKTKIISNRGENSCKATGQVCHALCSPEGCWGPEPRDCVSCRNVSRGRECVDKCNLLEGEPREFVENSECIQCCIQCAHYIDGPHCVKTCPAGVMGENNTLVWKYADAGHVCHLCHPNCTYGCTGPGLEGCPTNGPKIPSAAAHHHHHH

SEQ ID NO: 66 - protein, 636 aa, synthetic construct
DAAQPALEEKKVCQGTSNKLTQLGTFEDHFLSLQRMFNNCEVVLGNLEITYVQRNYDLSFLKTIQEVAGYVLIALNTVERIPLENLQIIRGNMYYENSYALAVLSNYDANKTGLKELPMRNLQEILHGAVRFSNNPALCNVESIQWRDIVSSDFLSNMSMDFQNHLGSCQKCDPSCPNGSCWGAGEENCQKLTKIICAQQCSGRCRGKSPSDCCHNQCAAGCTGPRESDCLVCRKFRDEATCKDTCPPLMLYNPTTYQMDVNPEGKYSFGATCVKKCPRNYVVTDHGSCVRACGADSYEMEEDGVRKCKKCEGPCRKVCNGIGIGEFKDSLSINATNIKHFKNCTSISGDLHILPVAFRGDSFTHTPPLDPQELDILKTVKEITGFLLIQAWPENRTDLHAFENLEIIRGRTKQHGQFSLAVVSLNITSLGLRSLKEISDGDVIISRNKNLCYANTINWKKLFGTSGQKTKIISNRGENSCKATGQVCHALCSPEGCWGPEPRDCVSCRNVSRGRECVDKCNLLEGEPREFVENSECIQCHPECLPQAMNITCTGRGPDNCIQCAHYIDGPHCVKTCPAGVMGENNTLVWKYADAGHVCHLCHPNCTYGCTGPGLEGCPTNGPKIPSAAAHHHHHH

SEQ ID NO: 67 - protein, 636 aa, synthetic construct
DAAQPALEEKKVCQGTSNKLTQLGTFEDHFLSLQRMFNNCEVVLGNLEITYVQRNYDLSFLKTIQEVAGYVLIALNTVERIPLENLQIIRGNMYYENSYALAVLSNYDANKTGLKELPMRNLQEILHGAVRFSNNPALCNVESIQWRDIVSSDFLSNMSMDFQNHLGSCQKCDPSCPNGSCWGAGEENCQKLTKIICAQQCSGRCRGKSPSDCCHNQCAAGCTGPRESDCLVCRKFRDEATCKDTCPPLMLYNPTTYQMDVNPEGKYSFGATCVKKCPRNYVVTDHGSCVRACGADSYEMEEDGVRKCKKCEGPCRKVCNGIGIGEFKDSLSINATNIKHFKNCTSISGDLHILPVAFRGDSFTHTPPLDPQELDILKTVKEITGFLLIQAWPENRTDLHAFENLEIIRGRTKQHGQFSLAVVSLNITSLGLRSLKEISDGDVIISGNKNLCYANTINWKKLFGTSGQKTKIIRNRGENSCKATGQVCHALCSPEGCWGPEPRDCVSCRNVSRGRECVDKCNLLEGEPREFVENSECIQCHPECLPQAMNITCTGRGPDNCIQCAHYIDGPHCVKTCPAGVMGENNTLVWKYADAGHVCHLCHPNCTYGCTGPGLEGCPTNGPKIPSAAAHHHHHH

SEQ ID NO: 68 - protein, 636 aa, synthetic construct
DAAQPALEEKKVCQGTSNKLTQLGTFEDHFLSLQRMFNNCEVVLGNLEITYVQRNYDLSFLKTIQEVAGYVLIALNTVERIPLENLQIIRGNMYYENSYALAVLSNYDANKTGLKELPMRNLQEILHGAVRFSNNPALCNVESIQWRDIVSSDFLSNMSMDFQNHLGSCQKCDPSCPNGSCWGAGEENCQKLTKIICAQQCSGRCRGKSPSDCCHNQCAAGCTGPRESDCLVCRKFRDEATCKDTCPPLMLYNPTTYQMDVNPEGKYSFGATCVKKCPRNYVVTDHGSCVRACGADSYEMEEDGVRKCKKCEGPCRKVCNGIGIGEFKDSLSINATNIKHFKNCTSISGDLHILPVAFRGDSFTHTPPLDPQELDILKTVKEITGFLLIQAWPENRTDLHAFENLEIIRGRTKQHGQASLAVVSLNITSLGLRSLKEISDGDVAISGNKNLCYANTINWKKLFGTSGQKTKIISNRGENSCKATGQVCHALCSPEGCWGPEPRDCVSCRNVSRGRECVDKCNLLEGEPREFVENSECIQCHPECLPQAMNITCTGRGPDNCIQCAHYIDGPHCVKTCPAGVMGENNTLVWKYADAGHVCHLCHPNCTYGCTGPGLEGCPTNGPKIPSAAAHHHHHH

SEQ ID NO: 69 - protein, 621 aa, Homo sapiens [sequence omitted]

SEQ ID NO: 70 - protein, 623 aa, Mus musculus
LEEKKVCQGTSNRLTQLGTFEDHFLSLQRMYNNCEVVLGNLEITYVQRNYDLSFLKTIQEVAGYVLIALNTVERIPLENLQIIRGNALYENTYALAILSNYGTNRTGLRELPMRNLQEILIGAVRFSNNPILCNMDTIQWRDIVQNVFMSNMSMDLQSHPSSCPKCDPSCPNGSCWGGGEENCQKLTKIICAQQCSHRCRGRSPSDCCHNQCAAGCTGPRESDCLVCQKFQDEATCKDTCPPLMLYNPTTYQMDVNPEGKYSFGATCVKKCPRNYVVTDHGSCVRACGPDYYEVEEDGIRKCKKCDGPCRKVCNGIGIGEFKDTLSINATNIKHFKYCTAISGDLHILPVAFKGDSFTRTPPLDPRELEILKTVKEITGFLLIQAWPDNWTDLHAFENLEIIRGRTKQHGQFSLAVVGLNITSLGLRSLKEISDGDVIISGNRNLCYANTINWKKLFGTPNQKTKIMNNRAEKDCKAVNHVCNPLCSSEGCWGPEPRDCVSCQNVSRGRECVEKCNILEGEPREFVENSECIQCHPECLPQAMNITCTGRGPDNCIQCAHYIDGPHCVKTCPAGIMGENNTLVWKYADANNVCHLCHANCTYGCAGPGLQGCEVWPSGPKIPS

SEQ ID NO: 71 - protein, 5 aa, synthetic construct
SYGMH

SEQ ID NO: 72 - protein, 17 aa, synthetic construct
FIRYDGSNKYYADSVKG

SEQ ID NO: 73 - protein, 11 aa, synthetic construct
DGNSGYDSMDY

SEQ ID NO: 74 - protein, 120 aa, synthetic construct
QVQLVQSGGGVVQPGGSLRLSCAASGFTFSSYGMHWVRQAPGKGLEWVAFIRYDGSNKYYADSVKGRFTISRDNSKNTLYLQMNSLRAEDTAVYYCAKDGNSGYDSMDYWGQGTLVTVSS

SEQ ID NO: 75 - protein, 120 aa, synthetic construct
QVQLQESGGGVVQPGGSLRLSCAASGFTFSSYGMHWVRQAPGKGLEWVAFIRYDGSNKYYADSVKGRFTISRDNSKNTLYLQMNSLRAEDTAVYYCAKDGNSGYDSMDYWGQGTLVTVSS

SEQ ID NO: 76 - protein, 13 aa, synthetic construct
SGVSSNIGRNYVY

SEQ ID NO: 77 - protein, 13 aa, synthetic construct
SGGSSNVGRNGVN

SEQ ID NO: 78 - protein, 7 aa, synthetic construct
ATHQRPS

SEQ ID NO: 79 - protein, 7 aa, synthetic construct
YDAFLSS

SEQ ID NO: 80 - protein, 11 aa, synthetic construct
AAWDDGVTGWV

SEQ ID NO: 81 - protein, 11 aa, synthetic construct
ASWDDSLTGWV

SEQ ID NO: 82 - protein, 11 aa, synthetic construct
AAWDDSLYSWV

SEQ ID NO: 83 - protein, 110 aa, synthetic construct
QPVLTQSPSASGTPGQRVTISCSGVSSNIGRNYVYWYQQFPGTAPKLLIYATHQRPSGVPDRFSGSKSGTSASLAISGLRSEDEANYYCAAWDDGVTGWVFGGGTKLTVL

SEQ ID NO: 84 - protein, 110 aa, synthetic construct
QSVLTQPPSVSGAPGQRVTISCSGGSSNVGRNGVNWFQHLPEKAPKLLIYYDAFLSSGVSDRFSGSKSGTSASLAIRGLQSEDEADYYCASWDDSLTGWVFGGGTKLTVL

SEQ ID NO: 85 - protein, 110 aa, synthetic construct
QSVLTQPPSVSGAPGQRVTISCSGGSSNVGRNGVNWFQHLPEKAPKLLIYYDAFLSSGVSDRFSGSKSGTSASLAIRGLQSDDEADYYCAAWDDSLYSWVFGGGTNLTVL

SEQ ID NO: 86 - protein, 13 aa, synthetic construct
  VARIANT 3: note = X is V or G
  VARIANT 7: note = X is I or V
  VARIANT 11: note = X is Y or G
  VARIANT 13: note = X is Y or N
SGXSSNXGRNXVX

SEQ ID NO: 87 - skipped

SEQ ID NO: 88 - protein, 11 aa, synthetic construct
  VARIANT 2: note = X is A or S
  VARIANT 6: note = X is G or S
  VARIANT 7: note = X is V or L
  VARIANT 8: note = X is T or Y
  VARIANT 9: note = X is G or S
AXWDDXXXXWV

SEQ ID NO: 89 - protein, 108 aa, synthetic construct
QPGLTQPPSVSVAPGKTARITCGGNNIGSKSVHWYQQKPGQAPVLVIYYDSDRPSGIPERFSGSNSGNTATLTISRVEAGDEADYYCQVWDSSSDHRVFGGGTKLTVL

SEQ ID NO: 90 - protein, 118 aa, synthetic construct
QVQLQESGPGLVKPSQTLSLTCTVSGGSISSGVYYWSWIRQHPGKGLEWIGYIYYSGSTYYNPSLKSRVTISVDTSKNQFSLKLSSVTAADTAVYYCARDLGGWFDPWGQGTLVTVSS

SEQ ID NO: 91 - protein, 106 aa, Homo sapiens
DFTPPTVKILQSSCDGGGHFPPTIQLLCLVSGYTPGTINITWLEDGQVMDVDLSTASTTQEGELASTQSELTLSQKHWLSDRTYTCQVTYQGHTFEDSTKKCADSN

SEQ ID NO: 92 - protein, 495 aa, synthetic construct
QVQLVQSGGGVVQPGGSLRLSCAASGFTFSSYGMHWVRQAPGKGLEWVAFIRYDGSNKYYADSVKGRFTISRDNSKNTLYLQMNSLRAEDTAVYYCAKDGNSGYDSMDYWGQGTLVTVSSGSASAPKLEEGEFSEARVQSVLTQPPSVSGAPGQRVTISCSGGSSNVGRNGVNWFQHLPEKAPKLLIYYDAFLSSGVSDRFSGSKSGTSASLAIRGLQSDDEADYYCAAWDDSLYSWVFGGGTNLTVLGQPKAAPSVTLFPPSSAAASDKTHTCPPCPAPELLGGPSVFLFPPKPKDTLMISRTPEVTCVVVDVSHEDPEVKFNWYVDGVEVHNAKTKPREEQYNSTYRVVSVLTVLHQDWLNGKEYKCKVSNKALPAPIEKTISKAKGQPREPQVYTLPPSRDELTKNQVSLTCLVKGFYPSDIAVEWESNGQPENNYKTTPPVLDSDGSFFLYSKLTVDKSRWQQGNVFSCSVMHEALHNHYTQKSLSLSPGK

SEQ ID NO: 93 - protein, 495 aa, synthetic construct
QVQLQESGGGVVQPGGSLRLSCAASGFTFSSYGMHWVRQAPGKGLEWVAFIRYDGSNKYYADSVKGRFTISRDNSKNTLYLQMNSLRAEDTAVYYCAKDGNSGYDSMDYWGQGTLVTVSSGSASAPKLEEGEFSEARVQSVLTQPPSVSGAPGQRVTISCSGGSSNVGRNGVNWFQHLPEKAPKLLIYYDAFLSSGVSDRFSGSKSGTSASLAIRGLQSEDEADYYCASWDDSLTGWVFGGGTKLTVLGQPKAAPSVTLFPPSSAAASDKTHTCPPCPAPELLGGPSVFLFPPKPKDTLMISRTPEVTCVVVDVSHEDPEVKFNWYVDGVEVHNAKTKPREEQYNSTYRVVSVLTVLHQDWLNGKEYKCKVSNKALPAPIEKTISKAKGQPREPQVYTLPPSRDELTKNQVSLTCLVKGFYPSDIAVEWESNGQPENNYKTTPPVLDSDGSFFLYSKLTVDKSRWQQGNVFSCSVMHEALHNHYTQKSLSLSPGK

SEQ ID NO: 94 - protein, 106 aa, synthetic construct
DFTPPTVKILQSSCDGGGHFPPTIQLLCLVSGYTPGTINITWLEDGQVMDVDLSTASTTQEGELASTQSELTLSQKHWLSDRTYTCQVTYQGHTFEDSTKKSADSN

SEQ ID NO: 95 - protein, 106 aa, synthetic construct
DFTPPTVKILQSSSDGGGHFPPTIQLLCLVSGYTPGTIQITWLEDGQVMDVDLSTASTTQEGELASTQSELTLSQKHWLSDRTYTCQVTYQGHTFEDSTKKCADSN

SEQ ID NO: 96 - protein, 122 aa, synthetic construct
QVQLVQSGAEVKKPGSSVKVSCKASGGTFSGYTMNWVRQAPGQGLEWMGLINPYKGVSTYNGKFKDRVTITADKSTSTAYMELSSLRSEDTAVYYCARSGYYGDSDWYFDVWGQGTLVTVSS

SEQ ID NO: 97 - protein, 109 aa, synthetic construct
DIQMTQSPSSLSASVGDRVTITCRASQDIRNYLNWYQQKPGKAPKLLIYYTSRLHSGVPSRFSGSGSGTDFTFTISSLQPEDIATYYCQQGNTLPWTFGQGTKLEIKRT

SEQ ID NO: 98 - protein, 8 aa, synthetic construct
GFTFSSYG

SEQ ID NO: 99 - protein, 8 aa, synthetic construct
IRYDGSNK

SEQ ID NO: 100 - protein, 13 aa, synthetic construct
AKDGNSGYDSMDY

SEQ ID NO: 101 - protein, 7 aa, synthetic construct
GFTFSSY

SEQ ID NO: 102 - protein, 6 aa, synthetic construct
RYDGSN

SEQ ID NO: 103 - protein, 11 aa, synthetic construct
DGNSGYDSMDY

SEQ ID NO: 104 - protein, 6 aa, synthetic construct
SSYGMH

SEQ ID NO: 105 - protein, 13 aa, synthetic construct
WVAFIRYDGSNKY

SEQ ID NO: 106 - protein, 10 aa, synthetic construct
DGNSGYDSMD

SEQ ID NO: 107 - protein, 8 aa, synthetic construct
SSNIGRNY

SEQ ID NO: 108 - protein, 8 aa, synthetic construct
SSNVGRNG

SEQ ID NO: 109-110 - skipped (2 entries)

SEQ ID NO: 111 - protein, 9 aa, synthetic construct
VSSNIGRNY

SEQ ID NO: 112 - protein, 9 aa, synthetic construct
GSSNVGRNG

SEQ ID NO: 113 - protein, 8 aa, synthetic construct
WDDGVTGW

SEQ ID NO: 114 - protein, 8 aa, synthetic construct
WDDSLTGW

SEQ ID NO: 115 - protein, 8 aa, synthetic construct
WDDSLYSW

SEQ ID NO: 116 - protein, 8 aa, synthetic construct
IGRNYVYW

SEQ ID NO: 117 - protein, 8 aa, synthetic construct
VGRNGVNW

SEQ ID NO: 118 - protein, 10 aa, synthetic construct
LLIYATHQRP

SEQ ID NO: 119 - protein, 10 aa, synthetic construct
LLIYYDAFLS

SEQ ID NO: 120 - protein, 116 aa, synthetic construct
EVQLVESGGGLVQPGKSLKLSCEASGFTFSGYGMHWVRQAPGRGLESVAYITSSSINIKYADAVKGRFTVSRDNAKNLLFLQMNILKSEDTAMYYCARFDWDKNYWGQGTMVTVSS

SEQ ID NO: 121 - protein, 109 aa, synthetic construct
DIQMTQSPSSLPASLGDRVTINCQASQDISNYLNWYQQKPGKAPKLLIYYTNKLADGVPSRFSGSGSGRDSSFTISSLESEDIGSYYCQQYYNYPWTFGPGTKLEIKRT